European Patent Application EP 4 810 029 A1, published September 23, 2026. Title: 一种含核酸构建体的药物组合物及其医药用途. Applicant: 上海瑞宏迪医药有限公司. Application CN. The sequence listing filed with the application follows.

SEQUENCE LISTING (132 sequences)

SEQ ID NO: 1 - DNA, 517 bp, synthetic construct
  source 1..517: mol_type = other DNA; note = B1 (ACTG1 3'UTR)
ccgactacctcatgaagatcctcactgagcgaggctacagcttcaccaccacggccgagcgggaaatcgtgcgcgacatcaaggagaagctgtgctacgtcgccctggacttcgagcaggagatggccaccgccgcatcctcctcttctctggagaagagctacgagctgcccgatggccaggtcatcaccattggcaatgagcggttccggtgtccggaggcgctgttccagccttccttcctgggtatggaatcttgcggcatccacgagaccaccttcaactccatcatgaagtgtgacgtggacatccgcaaagacctgtacgccaacacggtgctgtcgggcggcaccaccatgtacccgggcattgccgacaggatgcagaaggagatcaccgccctggcgcccagcaccatgaagatcaagatcatcgcacccccagagcgcaagtactcggtgtggatcggtggctccatcctggcctcactgtccaccttccagcagatgtggattag

SEQ ID NO: 2 - DNA, 282 bp, synthetic construct
  source 1..282: mol_type = other DNA; note = B2 (ATP6V0B)
atgatatgtgtgggtggggccgtgcctcacttttatttattgctggttttcctgggacagctggagctgtgtcccttagcctttcagaggcttggtgttcagggccctccctgcactcccctcttgctgcgtgttgatttggaggcactgcagtccaggccgagtcctcagtgcggggagcaggctgctgctgctgactctgtgcagctgcgcacctgtgtcccccacctccaccctcaacccatcttcctagtgtttgtgaaataaacttggtatttgtct

SEQ ID NO: 3 - DNA, 308 bp, synthetic construct
  source 1..308: mol_type = other DNA; note = B3 (ATP6V0B)
gttgaagaacttctctctaccgagcagcccgtaaccccctttttctccctcactgctgcaggagtctgctacaccatttttgatttgggcttccgctttgatgtggcatggttcctgacggagacttcgcccttcatgtggtccaacctgggcattggcctagctatctccctgtctgtggttggggcagcctggggcatctatattaccggctcctccatcattggtggaggagtgaaggcccccaggatcaagaccaagaacctggtcagcatcatcttctgtgaggctgtggccatctacggcat

SEQ ID NO: 4 - DNA, 226 bp, synthetic construct
  source 1..226: mol_type = other DNA; note = B4 (ATP6V0E1 3'UTR)
ggaagaagacatgctctacagtgctcagtctttgaggtgactatgcttgtgacctttcttatcagtatggtcaggcagtcagagtttgccttgactttttctcacattttatggccattttaacacgtggcaagggcaagctgctgaatgcaaacacgatctgaagagcagaaataaaattggaacttaagccttagcttacctaaatctcattaagattcttttt

SEQ ID NO: 5 - DNA, 461 bp, synthetic construct
  source 1..461: mol_type = other DNA; note = B5 (ATP6V0E1 3'UTR)
atgcaaaatcacctccaaaccagaccacttttcttgacttgcctgttttggccattagctgccttaaacgttaacagcacatttgaatgccttattctacaatgcagcgtgttttcctttgccttttttgcactttggtgaattacgtgcctccataacctgaactgtgccgactccacaaaacgattatgtactcttctgagatagaagatgctgttcttctgagagatacgttactctctccttggaatctgtggatttgaagatggctcctgccttctcacgtgggaatcagtgaagtgtttagaaactgctgcaagacaaacaagactccagtggggtggtcagtaggagagcacgttcagagggaagagccatctcaacagaatcgcaccaaactatactttcaggatgaatttcttctttctgccatcttttggaataaatattttcctcctttc

SEQ ID NO: 6 - DNA, 499 bp, synthetic construct
  source 1..499: mol_type = other DNA; note = B6 (CFL1 3'UTR)
gccccttctggccccctgcctggagcatctggcagccccacacctgcccttgggggttgcaggctgcccccttcctgccagaccggaggggctggggggatcccagcagggggagggcaatcccttcaccccagttgccaaacagaccccccaccccctggattttccttctccctccatcccttgacggttctggccttcccaaactgcttttgatcttttgattcctcttgggctgaagcagaccaagttccccccaggcaccccagttgtgggggagcctgtattttttttaacaacatccccattccccacctggtcctcccccttcccatgctgccaacttctaaccgcaatagtgactctgtgcttgtctgtttagttctgtgtataaatggaatgttgtggagatgacccctccctgtgccggctggttcctctcccttttcccctggtcacggctactcatggaagcaggaccagtaagggaccttcgatt

SEQ ID NO: 7 - DNA, 282 bp, synthetic construct
  source 1..282: mol_type = other DNA; note = B7 (CFL1 3'UTR)
gccccttctggccccctgcctggagcatctggcagccccacacctgcccttgggggttgcaggctgcccccttcctgccagaccggaggggctggggggatcccagcagggggagggcaatcccttcaccccagttgccaaacagaccccccaccccctggattttccttctccctccatcccttgacggttctggccttcccaaactgcttttgatcttttgattcctcttgggctgaagcagaccaagttccccccaggcaccccagttgtgggggagcc

SEQ ID NO: 8 - DNA, 361 bp, synthetic construct
  source 1..361: mol_type = other DNA; note = B8 (CFL1 3'UTR)
gccccttctggccccctgcctggagcatctggcagccccacacctgcccttgggggttgcaggctgcccccttcctgccagaccggaggggctggggggatcccagcagggggagggcaatcccttcaccccagttgccaaacagaccccccaccccctggattttccttctccctccatcccttgacggttctggccttcccaaactgcttttgatcttttgattcctcttgggctgaagcagaccaagttccccccaggcaccccagttgtgggggagcctgtattttttttaacaacatccccattccccacctggtcctcccccttcccatgctgccaacttctaaccgcaatagtg

SEQ ID NO: 9 - DNA, 128 bp, synthetic construct
  source 1..128: mol_type = other DNA; note = B9 (COX4I1 3'UTR)
gagatgctggcctgcgcctgcacctgcgcctggctctgtcaccgccatgcaactccatgcctatttactggaaacctgttatgccaaacagttgtaccactgctaataaatgaccagtttacctgaaa

SEQ ID NO: 10 - DNA, 319 bp, synthetic construct
  source 1..319: mol_type = other DNA; note = B10 (COX4I1 3'UTR)
agggacccacaggcgcgcccagcagctctcggaagcgttgtatcgcattaagttcaaggagagctttgctgagatgaacaggggctcgaacgagtggaagacggttgtgggcggtgccatgttcttcatcggtttcaccgcgctcgttatcatgtggcagaagcactatgggcttagcctccaagtgggactacgaaaagaacgagtggaagaagtgagagatgctggcctgcgcctgcacctgcgcctggctctgtcaccgccatgcaactccatgcctatttactggaaacctgttatgccaaacagttgtaccact

SEQ ID NO: 11 - DNA, 303 bp, synthetic construct
  source 1..303: mol_type = other DNA; note = B11 (COX4I1 3'UTR)
agaggaccttctgcttttagcttattttgttgctaactttttacaaacaaagggctaattttaaaatgtcagtgttgtcagtggtcagaaaccgtgtgtttgagcgggtgttgagtggcaggtggctctgctgacctggtggctggtgtgtcgggaggatttaacctgtgtgagggattggcctagaaacaacctgttgagatagtcttgccccataacctgtctcacaccgtagtgtacggccccctcccgcaaagctttgacaaagagtgggtggccaagcagaccaagaggatgctggac

SEQ ID NO: 12 - DNA, 232 bp, synthetic construct
  source 1..232: mol_type = other DNA; note = B12 (CTSB 3'UTR)
tctgccgtgggcctgtcgtgccagtcctgggggcgagatcgggagaatcacgtcctggaactgcatgttcttgcgactcttgggacttcatcttaacttctcgctgccccagccatgttttcaaccatggcatccctcccccaattagttccctgtcatcctcgtcaaccttctctgtaagtgcctggtaagcttgcccttgcttaagaactcaaaacatagctgtgctcta

SEQ ID NO: 13 - DNA, 115 bp, synthetic construct
  source 1..115: mol_type = other DNA; note = B13 (FAM166A 3'UTR)
aaatgctttaatggtggtgtctgtacagcatggatgtggacagggaaaacagcaagtgcacacagtgggacaggccacaggacaggctgggagtgaataaagagttcacactgct

SEQ ID NO: 14 - DNA, 196 bp, synthetic construct
  source 1..196: mol_type = other DNA; note = B14 (NDUFB9 3'UTR)
tatctaagtgtatcaatttaacatttataatcaccttacaagtaagttaaagtgcattccctggtcgttttggctttgtctttgattttgcttcagatctccttctctttagtcctttgtctgacttttttgccttcttgctatactttccctcaacctgcctctccactattttcttaggcatttttcagtcatg

SEQ ID NO: 15 - DNA, 54 bp, synthetic construct
  source 1..54: mol_type = other DNA; note = A1 (ACTG1 5'UTR)
ctctcgcactctgttcttccgccgctccgccgtcgcgtttctctgccggtcgca

SEQ ID NO: 16 - DNA, 185 bp, synthetic construct
  source 1..185: mol_type = other DNA; note = A2 (ATP6V0B 5'UTR)
gggcgggcggacagactgcgggacggacggtggacgctgggacgcgtttgtagctccggccccgccgttccgacccccgccgccgtcgccgccatgacggggctagcactgctctactccggggtcttcgtggccttctgggcctgcgcgctggccgtgggttcctgacggagacttcgcccttc

SEQ ID NO: 17 - DNA, 81 bp, synthetic construct
  source 1..81: mol_type = other DNA; note = A3 (ATP6V0B 5'UTR)
agactgcgggacggacggtggacgctgggacgcgtttgtagctccggccccgccgttccgacccccgccgccgtcgccgcc

SEQ ID NO: 18 - DNA, 30 bp, synthetic construct
  source 1..30: mol_type = other DNA; note = A4 (ATP6V0E1 5'UTR)
ggggtaggggttggcgctcaggcggcgacc

SEQ ID NO: 19 - DNA, 80 bp, synthetic construct
  source 1..80: mol_type = other DNA; note = A5 (ATP6V0E1 5'UTR)
gtcacgcggtcagctattgacacttcctggtgggatccgagtgaggcgacggggtaggggttggcgctcaggcggcgacc

SEQ ID NO: 20 - DNA, 234 bp, synthetic construct
  source 1..234: mol_type = other DNA; note = A6 (CFL1 5'UTR)
ggccggcgggaagactccgttacccagcgagcgaggcggcggcgcagggccagcggactccatttcccgtcggctcgcggtgggagcgccggaagcccgccccacccctcattgtgcggctcctactaaacggaaggggccgggagaggccgcgttcagtcgggtcccggcagcggctgcagcgctctcgtcttctgcggctctcggtgccctctccttttcgtttccggaaac

SEQ ID NO: 21 - DNA, 128 bp, synthetic construct
  source 1..128: mol_type = other DNA; note = A7 (CFL1 5'UTR)
ctcctggctcgggcaccccgaagcacgacgcagagtaggaagagtttaaagacctcgaggcctctgggcacttgagtttggcctccggtgtggctgtctctgatggtgtcatcaaggtgttcaacgac

SEQ ID NO: 22 - DNA, 151 bp, synthetic construct
  source 1..151: mol_type = other DNA; note = A8 (CFL1 5'UTR)
acgtggccggcttcttctgcagttccggggagtttgggggaccagatttaccttggattgcccctccctctcctggctcgggcaccccgaagcacgacgcagagcctccggtgtggctgtctctgatggtgtcatcaaggtgttcaacgac

SEQ ID NO: 23 - DNA, 70 bp, synthetic construct
  source 1..70: mol_type = other DNA; note = A9 (COX4I1 5'UTR)
gcggccttgctctcttccggtcgcgggacaccgggtgtagagggcggtcgcggcgggcagtggcggcaga

SEQ ID NO: 24 - DNA, 46 bp, synthetic construct
  source 1..46: mol_type = other DNA; note = A10 (COX4I1 5'UTR)
gggacaccgggtgtagagggcggtcgcggcgggcagtggcggcaga

SEQ ID NO: 25 - DNA, 71 bp, synthetic construct
  source 1..71: mol_type = other DNA; note = A11 (COX4I1 5'UTR)
cgcggccttgctctcttccggtcgcgggacaccgggtgtagagggcggtcgcggcgggcagtggcggcaga

SEQ ID NO: 26 - DNA, 137 bp, synthetic construct
  source 1..137: mol_type = other DNA; note = A12 (CTSB 5'UTR)
ggccggggctggcccaggctacggcggctgcagggctccggcaaccgctccggcaacgccaaccgctccgctgcgcgcaggctgggctgcaggctctcggctgcagcgctgggtggatctaggatccggcttccaac

SEQ ID NO: 27 - DNA, 55 bp, synthetic construct
  source 1..55: mol_type = other DNA; note = A13 (FAM166A 5'UTR)
aagggagctggatgccgggagggactggagccagcaaggccagagtgaaagcaaa

SEQ ID NO: 28 - DNA, 56 bp, synthetic construct
  source 1..56: mol_type = other DNA; note = A14 (NDUFB9 5'UTR)
gcagcaggcgtgcagtttcccggctctccgcgcggccggggaaggtcagcgccgta

SEQ ID NO: 29 - DNA, 68 bp, synthetic construct
  source 1..68: mol_type = other DNA; note = A15 (CHCHD10 5'UTR)
ggcatttgtccccgcgacagcaccgctgccgccgtctctaaggtcgcccgggtcccaccgccgccacc

SEQ ID NO: 30 - DNA, 46 bp, synthetic construct
  source 1..46: mol_type = other DNA; note = A16 (CHCHD10 5'UTR)
ccgctgccgccgtctctaaggtcgcccgggtcccaccgccgccacc

SEQ ID NO: 31 - DNA, 41 bp, synthetic construct
  source 1..41: mol_type = other DNA; note = A17 (SLC38A2 5'UTR)
atgtcttttttgtgtgtttgttttcatggtattcctatgaa

SEQ ID NO: 32 - DNA, 48 bp, synthetic construct
  source 1..48: mol_type = other DNA; note = A18 (NDUFA11 5'UTR)
gcttcccgagctggcggggtccgtggtgcgggatcgagattgcgggct

SEQ ID NO: 33 - DNA, 69 bp, synthetic construct
  source 1..69: mol_type = other DNA; note = A19 (NDUFV3 5'UTR)
ggcggctgttcaggcgcgggtgcgcgcgcagctgctgtggccctgcttggtgcgcccgctgtcaccgcc

SEQ ID NO: 34 - DNA, 128 bp, synthetic construct
  source 1..128: mol_type = other DNA; note = A20 (PRDX5 5'UTR)
cgcgcctgcgcagtggaggcggcccaggcccgccttccgcagggtgtcgccgctgtgccgctagcggtgccccgcctgctgcggtggcaccagccaggaggcggagtggaagtggccgtggggcgggt

SEQ ID NO: 35 - DNA, 59 bp, synthetic construct
  source 1..59: mol_type = other DNA; note = A21 (GUK1 5'UTR)
cagcagatggggactagaggccgcactgctatccacagcctctcttctcacccccaggc

SEQ ID NO: 36 - DNA, 68 bp, synthetic construct
  source 1..68: mol_type = other DNA; note = A22 (GUK1 5'UTR)
gctggccgggctggctgcggccgccctgggccgggccccaccggacgcctctcttctcacccccaggc

SEQ ID NO: 37 - DNA, 96 bp, synthetic construct
  source 1..96: mol_type = other DNA; note = A23 (GUK1 5'UTR)
agaggtggccccggatgctgcggcgcccgctggccgggctggctgcggccgccctgggccgggccccaccggacgcctctcttctcacccccaggc

SEQ ID NO: 38 - DNA, 37 bp, synthetic construct
  source 1..37: mol_type = other DNA; note = A24 (IAH1 5'UTR)
tggctggcggccccgccccgccccgcccggctgctcc

SEQ ID NO: 39 - DNA, 59 bp, synthetic construct
  source 1..59: mol_type = other DNA; note = A25 (ABHD16A 5'UTR)
ggagggcggggccggcagggggacctgctgctggaagagcagcggcccgagccggggcc

SEQ ID NO: 40 - DNA, 132 bp, synthetic construct
  source 1..132: mol_type = other DNA; note = A26 (SLC25A39 5'UTR)
tttcggcgtcggcctaggtgcgctgcgagcgcgcgcggaccgcgcacaggcggcggagccggtatgggcccgcctgaccctgggcgccgcgccgcacgagcaccagcctagagccaggactgaagcttcaag

SEQ ID NO: 41 - DNA, 51 bp, synthetic construct
  source 1..51: mol_type = other DNA; note = A27 (ATPIF1 5'UTR)
cgagagactgcttgctgcggcagagacgccagaggtgcagctccagcagca

SEQ ID NO: 42 - DNA, 71 bp, synthetic construct
  source 1..71: mol_type = other DNA; note = A28 (ANAPC11 5'UTR)
cggagtttcgtcatgttggccaggcccatttgagatctttgaagatatcctcaacgtgaggctctgctgcc

SEQ ID NO: 43 - DNA, 55 bp, synthetic construct
  source 1..55: mol_type = other DNA; note = A29 (ANAPC11 5'UTR)
gggcgcggcttcggcgggcggcagccgctgcagacgagctgcgggctctgctgcc

SEQ ID NO: 44 - DNA, 48 bp, synthetic construct
  source 1..48: mol_type = other DNA; note = A30 (CCDC12 5'UTR)
gcctgcgcgatgcaagacgggagaaaaggaggggcgtacgcgggcaag

SEQ ID NO: 45 - DNA, 132 bp, synthetic construct
  source 1..132: mol_type = other DNA; note = A31 (MRPL14 5'UTR)
atcgcgtccgccgggctgggcctggcgcgcaggcgctaggaagaggccgcgtggggcgaaggcggcgcttggctggtggggcccgcggcgggattttcccgggcggcgagagcggatctatcttgggatccc

SEQ ID NO: 46 - DNA, 27 bp, synthetic construct
  source 1..27: mol_type = other DNA; note = A32 (APOA1BP 5'UTR)
gccgggggcgcgcgctctgcgagctgg

SEQ ID NO: 47 - DNA, 43 bp, synthetic construct
  source 1..43: mol_type = other DNA; note = A33 (APOA1BP 5'UTR)
gccggggccgggccgggccgggggcgcgcgctctgcgagctgg

SEQ ID NO: 48 - DNA, 47 bp, synthetic construct
  source 1..47: mol_type = other DNA; note = Mod. 5'UTR
gggaaataagagagaaaagaagagtaagaagaaatataagagccacc

SEQ ID NO: 49 - DNA, 119 bp, synthetic construct
  source 1..119: mol_type = other DNA; note; note (original language) = a-globin 3'UTR
tgataataggctggagcctcggtggccatgcttcttgccccttgggcctccccccagcccctcctccccttcctgcacccgtacccccgtggtctttgaataaagtctgagtgggcggc

SEQ ID NO: 50 - RNA, 52 nt, synthetic construct
  source 1..52: mol_type = other RNA; note; note (original language) = a-1 globin 5'UTR
agacgaactagtattcttctggtccccacagactcagagagaacccgccacc

SEQ ID NO: 51 - DNA, 317 bp, synthetic construct
  source 1..317: mol_type = other DNA; note = haplogroup U8b1b1 mitochondrion 3'UTR
ctcgagctggtactgcatgcacgcaatgctagctgcccctttcccgtcctgggtaccccgagtctcccccgacctcgggtcccaggtatgctcccacctccacctgccccactcaccacctctgctagttccagacacctgctatactaatcgctagccgcgtcgctccccagggttggtcaatttcgtgccagccacaccgagacctggtccagagcccaagcacgccacacccccacgggaaacagcagtgattaacctttagcaataaacgaaagtttaactaacagcaatgcagctcaaaacgcttagcctag

SEQ ID NO: 52 - DNA, 110 bp, synthetic construct
  source 1..110: mol_type = other DNA; note = A30L70 PolyA
aaaaaaaaaaaaaaaaaaaaaaaaaaaaaagcatatgactaaaaaaaaaaaaaaaaaaaaaaaaaaaaaaaaaaaaaaaaaaaaaaaaaaaaaaaaaaaaaaaaaaaaaa

SEQ ID NO: 53 - DNA, 2014 bp, synthetic construct
  source 1..2014: mol_type = other DNA; note; note (original language) = 5'UTR-Fluc-a globin 3'UTR-120A (Mod.-120A)
gggaaataagagagaaaagaagagtaagaagaaatataagagccaccatggaagacgccaaaaacataaagaaaggcccggcgccattctatccgctggaagatggaaccgctggagagcaactgcataaggctatgaagagatacgccctggttcctggaacaattgcttttacagatgcacatatcgaggtggacatcacttacgctgagtacttcgaaatgtccgttcggttggcagaagctatgaaacgatatgggctgaatacaaatcacagaatcgtcgtatgcagtgaaaactctcttcaattctttatgccggtgttgggcgcgttatttatcggagttgcagttgcgcccgcgaacgacatttataatgaacgtgaattgctcaacagtatgggcatttcgcagcctaccgtggtgttcgtttccaaaaaggggttgcaaaaaattttgaacgtgcaaaaaaagctcccaatcatccaaaaaattattatcatggattctaaaacggattaccagggatttcagtcgatgtacacgttcgtcacatctcatctacctcccggttttaatgaatacgattttgtgccagagtccttcgatagggacaagacaattgcactgatcatgaactcctctggatctactggtctgcctaaaggtgtcgctctgcctcatagaactgcctgcgtgagattctcgcatgccagagatcctatttttggcaatcaaatcattccggatactgcgattttaagtgttgttccattccatcacggttttggaatgtttactacactcggatatttgatatgtggatttcgagtcgtcttaatgtatagatttgaagaagagctgtttctgaggagccttcaggattacaagattcaaagtgcgctgctggtgccaaccctattctccttcttcgccaaaagcactctgattgacaaatacgatttatctaatttacacgaaattgcttctggtggcgctcccctctctaaggaagtcggggaagcggttgccaagaggttccatctgccaggtatcaggcaaggatatgggctcactgagactacatcagctattctgattacacccgagggggatgataaaccgggcgcggtcggtaaagttgttccattttttgaagcgaaggttgtggatctggataccgggaaaacgctgggcgttaatcaaagaggcgaactgtgtgtgagaggtcctatgattatgtccggttatgtaaacaatccggaagcgaccaacgccttgattgacaaggatggatggctacattctggagacatagcttactgggacgaagacgaacacttcttcatcgttgaccgcctgaagtctctgattaagtacaaaggctatcaggtggctcccgctgaattggaatccatcttgctccaacaccccaacatcttcgacgcaggtgtcgcaggtcttcccgacgatgacgccggtgaacttcccgccgccgttgttgttttggagcacggaaagacgatgacggaaaaagagatcgtggattacgtcgccagtcaagtaacaaccgcgaaaaagttgcgcggaggagttgtgtttgtggacgaagtaccgaaaggtcttaccggaaaactcgacgcaagaaaaatcagagagatcctcataaaggccaagaagggcggaaagatcgccgtggattacaaggatgacgacgataagtaagggcccaccggttgataataggctggagcctcggtggccatgcttcttgccccttgggcctccccccagcccctcctccccttcctgcacccgtacccccgtggtctttgaataaagtctgagtgggcggcctcgagccgcggaaaaaaaaaaaaaaaaaaaaaaaaaaaaaaaaaaaaaaaaaaaaaaaaaaaaaaaaaaaaaaaaaaaaaaaaaaaaaaaaaaaaaaaaaaaaaaaaaaaaaaaaaaaaaaaaaaaaaaaattattgtttaaacatttaaattctaga

SEQ ID NO: 54 - DNA, 2004 bp, synthetic construct
  source 1..2004: mol_type = other DNA; note; note (original language) = 5'UTR-Fluc-a globin 3'UTR-A30L70 (Mod.-A30L70)
gggaaataagagagaaaagaagagtaagaagaaatataagagccaccatggaagacgccaaaaacataaagaaaggcccggcgccattctatccgctggaagatggaaccgctggagagcaactgcataaggctatgaagagatacgccctggttcctggaacaattgcttttacagatgcacatatcgaggtggacatcacttacgctgagtacttcgaaatgtccgttcggttggcagaagctatgaaacgatatgggctgaatacaaatcacagaatcgtcgtatgcagtgaaaactctcttcaattctttatgccggtgttgggcgcgttatttatcggagttgcagttgcgcccgcgaacgacatttataatgaacgtgaattgctcaacagtatgggcatttcgcagcctaccgtggtgttcgtttccaaaaaggggttgcaaaaaattttgaacgtgcaaaaaaagctcccaatcatccaaaaaattattatcatggattctaaaacggattaccagggatttcagtcgatgtacacgttcgtcacatctcatctacctcccggttttaatgaatacgattttgtgccagagtccttcgatagggacaagacaattgcactgatcatgaactcctctggatctactggtctgcctaaaggtgtcgctctgcctcatagaactgcctgcgtgagattctcgcatgccagagatcctatttttggcaatcaaatcattccggatactgcgattttaagtgttgttccattccatcacggttttggaatgtttactacactcggatatttgatatgtggatttcgagtcgtcttaatgtatagatttgaagaagagctgtttctgaggagccttcaggattacaagattcaaagtgcgctgctggtgccaaccctattctccttcttcgccaaaagcactctgattgacaaatacgatttatctaatttacacgaaattgcttctggtggcgctcccctctctaaggaagtcggggaagcggttgccaagaggttccatctgccaggtatcaggcaaggatatgggctcactgagactacatcagctattctgattacacccgagggggatgataaaccgggcgcggtcggtaaagttgttccattttttgaagcgaaggttgtggatctggataccgggaaaacgctgggcgttaatcaaagaggcgaactgtgtgtgagaggtcctatgattatgtccggttatgtaaacaatccggaagcgaccaacgccttgattgacaaggatggatggctacattctggagacatagcttactgggacgaagacgaacacttcttcatcgttgaccgcctgaagtctctgattaagtacaaaggctatcaggtggctcccgctgaattggaatccatcttgctccaacaccccaacatcttcgacgcaggtgtcgcaggtcttcccgacgatgacgccggtgaacttcccgccgccgttgttgttttggagcacggaaagacgatgacggaaaaagagatcgtggattacgtcgccagtcaagtaacaaccgcgaaaaagttgcgcggaggagttgtgtttgtggacgaagtaccgaaaggtcttaccggaaaactcgacgcaagaaaaatcagagagatcctcataaaggccaagaagggcggaaagatcgccgtggattacaaggatgacgacgataagtaagggcccaccggttgataataggctggagcctcggtggccatgcttcttgccccttgggcctccccccagcccctcctccccttcctgcacccgtacccccgtggtctttgaataaagtctgagtgggcggcctcgagccgcggaaaaaaaaaaaaaaaaaaaaaaaaaaaaaagcatatgactaaaaaaaaaaaaaaaaaaaaaaaaaaaaaaaaaaaaaaaaaaaaaaaaaaaaaaaaaaaaaaaaaaaaaattattgtttaaacatttaaattctaga

SEQ ID NO: 55 - DNA, 2206 bp, synthetic construct
  source 1..2206: mol_type = other DNA; note; note (original language) = a-1-globin 5'UTR-Fluc-haplogroup U8b1b1 mitochondrion 3'UTR-A30L70 (BioN.)
agacgaactagtattcttctggtccccacagactcagagagaacccgccaccatggaagacgccaaaaacataaagaaaggcccggcgccattctatccgctggaagatggaaccgctggagagcaactgcataaggctatgaagagatacgccctggttcctggaacaattgcttttacagatgcacatatcgaggtggacatcacttacgctgagtacttcgaaatgtccgttcggttggcagaagctatgaaacgatatgggctgaatacaaatcacagaatcgtcgtatgcagtgaaaactctcttcaattctttatgccggtgttgggcgcgttatttatcggagttgcagttgcgcccgcgaacgacatttataatgaacgtgaattgctcaacagtatgggcatttcgcagcctaccgtggtgttcgtttccaaaaaggggttgcaaaaaattttgaacgtgcaaaaaaagctcccaatcatccaaaaaattattatcatggattctaaaacggattaccagggatttcagtcgatgtacacgttcgtcacatctcatctacctcccggttttaatgaatacgattttgtgccagagtccttcgatagggacaagacaattgcactgatcatgaactcctctggatctactggtctgcctaaaggtgtcgctctgcctcatagaactgcctgcgtgagattctcgcatgccagagatcctatttttggcaatcaaatcattccggatactgcgattttaagtgttgttccattccatcacggttttggaatgtttactacactcggatatttgatatgtggatttcgagtcgtcttaatgtatagatttgaagaagagctgtttctgaggagccttcaggattacaagattcaaagtgcgctgctggtgccaaccctattctccttcttcgccaaaagcactctgattgacaaatacgatttatctaatttacacgaaattgcttctggtggcgctcccctctctaaggaagtcggggaagcggttgccaagaggttccatctgccaggtatcaggcaaggatatgggctcactgagactacatcagctattctgattacacccgagggggatgataaaccgggcgcggtcggtaaagttgttccattttttgaagcgaaggttgtggatctggataccgggaaaacgctgggcgttaatcaaagaggcgaactgtgtgtgagaggtcctatgattatgtccggttatgtaaacaatccggaagcgaccaacgccttgattgacaaggatggatggctacattctggagacatagcttactgggacgaagacgaacacttcttcatcgttgaccgcctgaagtctctgattaagtacaaaggctatcaggtggctcccgctgaattggaatccatcttgctccaacaccccaacatcttcgacgcaggtgtcgcaggtcttcccgacgatgacgccggtgaacttcccgccgccgttgttgttttggagcacggaaagacgatgacggaaaaagagatcgtggattacgtcgccagtcaagtaacaaccgcgaaaaagttgcgcggaggagttgtgtttgtggacgaagtaccgaaaggtcttaccggaaaactcgacgcaagaaaaatcagagagatcctcataaaggccaagaagggcggaaagatcgccgtggattacaaggatgacgacgataagtaagggcccaccggctcgagctggtactgcatgcacgcaatgctagctgcccctttcccgtcctgggtaccccgagtctcccccgacctcgggtcccaggtatgctcccacctccacctgccccactcaccacctctgctagttccagacacctgctatactaatcgctagccgcgtcgctccccagggttggtcaatttcgtgccagccacaccgagacctggtccagagcccaagcacgccacacccccacgggaaacagcagtgattaacctttagcaataaacgaaagtttaactaacagcaatgcagctcaaaacgcttagcctagctcgagccgcggaaaaaaaaaaaaaaaaaaaaaaaaaaaaaagcatatgactaaaaaaaaaaaaaaaaaaaaaaaaaaaaaaaaaaaaaaaaaaaaaaaaaaaaaaaaaaaaaaaaaaaaaattattgtttaaacatttaaattctaga

SEQ ID NO: 56 - DNA, 2411 bp, synthetic construct
  source 1..2411: mol_type = other DNA; note = 5'UTR-Fluc- ACTG1 3'UTR-120A (B1)
gggaaataagagagaaaagaagagtaagaagaaatataagagccaccatggaagacgccaaaaacataaagaaaggcccggcgccattctatccgctggaagatggaaccgctggagagcaactgcataaggctatgaagagatacgccctggttcctggaacaattgcttttacagatgcacatatcgaggtggacatcacttacgctgagtacttcgaaatgtccgttcggttggcagaagctatgaaacgatatgggctgaatacaaatcacagaatcgtcgtatgcagtgaaaactctcttcaattctttatgccggtgttgggcgcgttatttatcggagttgcagttgcgcccgcgaacgacatttataatgaacgtgaattgctcaacagtatgggcatttcgcagcctaccgtggtgttcgtttccaaaaaggggttgcaaaaaattttgaacgtgcaaaaaaagctcccaatcatccaaaaaattattatcatggattctaaaacggattaccagggatttcagtcgatgtacacgttcgtcacatctcatctacctcccggttttaatgaatacgattttgtgccagagtccttcgatagggacaagacaattgcactgatcatgaactcctctggatctactggtctgcctaaaggtgtcgctctgcctcatagaactgcctgcgtgagattctcgcatgccagagatcctatttttggcaatcaaatcattccggatactgcgattttaagtgttgttccattccatcacggttttggaatgtttactacactcggatatttgatatgtggatttcgagtcgtcttaatgtatagatttgaagaagagctgtttctgaggagccttcaggattacaagattcaaagtgcgctgctggtgccaaccctattctccttcttcgccaaaagcactctgattgacaaatacgatttatctaatttacacgaaattgcttctggtggcgctcccctctctaaggaagtcggggaagcggttgccaagaggttccatctgccaggtatcaggcaaggatatgggctcactgagactacatcagctattctgattacacccgagggggatgataaaccgggcgcggtcggtaaagttgttccattttttgaagcgaaggttgtggatctggataccgggaaaacgctgggcgttaatcaaagaggcgaactgtgtgtgagaggtcctatgattatgtccggttatgtaaacaatccggaagcgaccaacgccttgattgacaaggatggatggctacattctggagacatagcttactgggacgaagacgaacacttcttcatcgttgaccgcctgaagtctctgattaagtacaaaggctatcaggtggctcccgctgaattggaatccatcttgctccaacaccccaacatcttcgacgcaggtgtcgcaggtcttcccgacgatgacgccggtgaacttcccgccgccgttgttgttttggagcacggaaagacgatgacggaaaaagagatcgtggattacgtcgccagtcaagtaacaaccgcgaaaaagttgcgcggaggagttgtgtttgtggacgaagtaccgaaaggtcttaccggaaaactcgacgcaagaaaaatcagagagatcctcataaaggccaagaagggcggaaagatcgccgtggattacaaggatgacgacgataagtaagggcccaccggccgactacctcatgaagatcctcactgagcgaggctacagcttcaccaccacggccgagcgggaaatcgtgcgcgacatcaaggagaagctgtgctacgtcgccctggacttcgagcaggagatggccaccgccgcatcctcctcttctctggagaagagctacgagctgcccgatggccaggtcatcaccattggcaatgagcggttccggtgtccggaggcgctgttccagccttccttcctgggtatggaatcttgcggcatccacgagaccaccttcaactccatcatgaagtgtgacgtggacatccgcaaagacctgtacgccaacacggtgctgtcgggcggcaccaccatgtacccgggcattgccgacaggatgcagaaggagatcaccgccctggcgcccagcaccatgaagatcaagatcatcgcacccccagagcgcaagtactcggtgtggatcggtggctccatcctggcctcactgtccaccttccagcagatgtggattagctcgagccgcggaaaaaaaaaaaaaaaaaaaaaaaaaaaaaaaaaaaaaaaaaaaaaaaaaaaaaaaaaaaaaaaaaaaaaaaaaaaaaaaaaaaaaaaaaaaaaaaaaaaaaaaaaaaaaaaaaaaaaaaattattgtttaaacatttaaattctaga

SEQ ID NO: 57 - DNA, 2027 bp, synthetic construct
  source 1..2027: mol_type = other DNA; note; note (original language) = ACTG1 5'UTR-Fluc-a globin 3'UTR-120A (A1)
ctctcgcactctgttcttccgccgctccgccgtcgcgtttctctgccggtcgcagccaccatggaagacgccaaaaacataaagaaaggcccggcgccattctatccgctggaagatggaaccgctggagagcaactgcataaggctatgaagagatacgccctggttcctggaacaattgcttttacagatgcacatatcgaggtggacatcacttacgctgagtacttcgaaatgtccgttcggttggcagaagctatgaaacgatatgggctgaatacaaatcacagaatcgtcgtatgcagtgaaaactctcttcaattctttatgccggtgttgggcgcgttatttatcggagttgcagttgcgcccgcgaacgacatttataatgaacgtgaattgctcaacagtatgggcatttcgcagcctaccgtggtgttcgtttccaaaaaggggttgcaaaaaattttgaacgtgcaaaaaaagctcccaatcatccaaaaaattattatcatggattctaaaacggattaccagggatttcagtcgatgtacacgttcgtcacatctcatctacctcccggttttaatgaatacgattttgtgccagagtccttcgatagggacaagacaattgcactgatcatgaactcctctggatctactggtctgcctaaaggtgtcgctctgcctcatagaactgcctgcgtgagattctcgcatgccagagatcctatttttggcaatcaaatcattccggatactgcgattttaagtgttgttccattccatcacggttttggaatgtttactacactcggatatttgatatgtggatttcgagtcgtcttaatgtatagatttgaagaagagctgtttctgaggagccttcaggattacaagattcaaagtgcgctgctggtgccaaccctattctccttcttcgccaaaagcactctgattgacaaatacgatttatctaatttacacgaaattgcttctggtggcgctcccctctctaaggaagtcggggaagcggttgccaagaggttccatctgccaggtatcaggcaaggatatgggctcactgagactacatcagctattctgattacacccgagggggatgataaaccgggcgcggtcggtaaagttgttccattttttgaagcgaaggttgtggatctggataccgggaaaacgctgggcgttaatcaaagaggcgaactgtgtgtgagaggtcctatgattatgtccggttatgtaaacaatccggaagcgaccaacgccttgattgacaaggatggatggctacattctggagacatagcttactgggacgaagacgaacacttcttcatcgttgaccgcctgaagtctctgattaagtacaaaggctatcaggtggctcccgctgaattggaatccatcttgctccaacaccccaacatcttcgacgcaggtgtcgcaggtcttcccgacgatgacgccggtgaacttcccgccgccgttgttgttttggagcacggaaagacgatgacggaaaaagagatcgtggattacgtcgccagtcaagtaacaaccgcgaaaaagttgcgcggaggagttgtgtttgtggacgaagtaccgaaaggtcttaccggaaaactcgacgcaagaaaaatcagagagatcctcataaaggccaagaagggcggaaagatcgccgtggattacaaggatgacgacgataagtaagggcccaccggttgataataggctggagcctcggtggccatgcttcttgccccttgggcctccccccagcccctcctccccttcctgcacccgtacccccgtggtctttgaataaagtctgagtgggcggcctcgagccgcggaaaaaaaaaaaaaaaaaaaaaaaaaaaaaaaaaaaaaaaaaaaaaaaaaaaaaaaaaaaaaaaaaaaaaaaaaaaaaaaaaaaaaaaaaaaaaaaaaaaaaaaaaaaaaaaaaaaaaaaattattgtttaaacatttaaattctaga

SEQ ID NO: 58 - RNA, 517 nt, synthetic construct
  source 1..517: mol_type = other RNA; note; note (original language) = B1 mRNA sequence (ACTG1 3'UTR)
ccgactacctcatgaagatcctcactgagcgaggctacagcttcaccaccacggccgagcgggaaatcgtgcgcgacatcaaggagaagctgtgctacgtcgccctggacttcgagcaggagatggccaccgccgcatcctcctcttctctggagaagagctacgagctgcccgatggccaggtcatcaccattggcaatgagcggttccggtgtccggaggcgctgttccagccttccttcctgggtatggaatcttgcggcatccacgagaccaccttcaactccatcatgaagtgtgacgtggacatccgcaaagacctgtacgccaacacggtgctgtcgggcggcaccaccatgtacccgggcattgccgacaggatgcagaaggagatcaccgccctggcgcccagcaccatgaagatcaagatcatcgcacccccagagcgcaagtactcggtgtggatcggtggctccatcctggcctcactgtccaccttccagcagatgtggattag

SEQ ID NO: 59 - RNA, 282 nt, synthetic construct
  source 1..282: mol_type = other RNA; note; note (original language) = B2 mRNA sequence (ATP6V0B 3'UTR)
atgatatgtgtgggtggggccgtgcctcacttttatttattgctggttttcctgggacagctggagctgtgtcccttagcctttcagaggcttggtgttcagggccctccctgcactcccctcttgctgcgtgttgatttggaggcactgcagtccaggccgagtcctcagtgcggggagcaggctgctgctgctgactctgtgcagctgcgcacctgtgtcccccacctccaccctcaacccatcttcctagtgtttgtgaaataaacttggtatttgtct

SEQ ID NO: 60 - RNA, 308 nt, synthetic construct
  source 1..308: mol_type = other RNA; note; note (original language) = B3 mRNA sequence (ATP6V0B 3'UTR)
gttgaagaacttctctctaccgagcagcccgtaaccccctttttctccctcactgctgcaggagtctgctacaccatttttgatttgggcttccgctttgatgtggcatggttcctgacggagacttcgcccttcatgtggtccaacctgggcattggcctagctatctccctgtctgtggttggggcagcctggggcatctatattaccggctcctccatcattggtggaggagtgaaggcccccaggatcaagaccaagaacctggtcagcatcatcttctgtgaggctgtggccatctacggcat

SEQ ID NO: 61 - RNA, 226 nt, synthetic construct
  source 1..226: mol_type = other RNA; note; note (original language) = B4 mRNA sequence (ATP6V0E1 3'UTR)
ggaagaagacatgctctacagtgctcagtctttgaggtgactatgcttgtgacctttcttatcagtatggtcaggcagtcagagtttgccttgactttttctcacattttatggccattttaacacgtggcaagggcaagctgctgaatgcaaacacgatctgaagagcagaaataaaattggaacttaagccttagcttacctaaatctcattaagattcttttt

SEQ ID NO: 62 - RNA, 461 nt, synthetic construct
  source 1..461: mol_type = other RNA; note; note (original language) = B5 mRNA sequence (ATP6V0E1 3'UTR)
atgcaaaatcacctccaaaccagaccacttttcttgacttgcctgttttggccattagctgccttaaacgttaacagcacatttgaatgccttattctacaatgcagcgtgttttcctttgccttttttgcactttggtgaattacgtgcctccataacctgaactgtgccgactccacaaaacgattatgtactcttctgagatagaagatgctgttcttctgagagatacgttactctctccttggaatctgtggatttgaagatggctcctgccttctcacgtgggaatcagtgaagtgtttagaaactgctgcaagacaaacaagactccagtggggtggtcagtaggagagcacgttcagagggaagagccatctcaacagaatcgcaccaaactatactttcaggatgaatttcttctttctgccatcttttggaataaatattttcctcctttc

SEQ ID NO: 63 - RNA, 499 nt, synthetic construct
  source 1..499: mol_type = other RNA; note; note (original language) = B6 mRNA sequence (CFL1 3'UTR)
gccccttctggccccctgcctggagcatctggcagccccacacctgcccttgggggttgcaggctgcccccttcctgccagaccggaggggctggggggatcccagcagggggagggcaatcccttcaccccagttgccaaacagaccccccaccccctggattttccttctccctccatcccttgacggttctggccttcccaaactgcttttgatcttttgattcctcttgggctgaagcagaccaagttccccccaggcaccccagttgtgggggagcctgtattttttttaacaacatccccattccccacctggtcctcccccttcccatgctgccaacttctaaccgcaatagtgactctgtgcttgtctgtttagttctgtgtataaatggaatgttgtggagatgacccctccctgtgccggctggttcctctcccttttcccctggtcacggctactcatggaagcaggaccagtaagggaccttcgatt

SEQ ID NO: 64 - RNA, 282 nt, synthetic construct
  source 1..282: mol_type = other RNA; note; note (original language) = B7 mRNA sequence (CFL1 3'UTR)
gccccttctggccccctgcctggagcatctggcagccccacacctgcccttgggggttgcaggctgcccccttcctgccagaccggaggggctggggggatcccagcagggggagggcaatcccttcaccccagttgccaaacagaccccccaccccctggattttccttctccctccatcccttgacggttctggccttcccaaactgcttttgatcttttgattcctcttgggctgaagcagaccaagttccccccaggcaccccagttgtgggggagcc

SEQ ID NO: 65 - RNA, 361 nt, synthetic construct
  source 1..361: mol_type = other RNA; note; note (original language) = B8 mRNA sequence (CFL1 3'UTR)
gccccttctggccccctgcctggagcatctggcagccccacacctgcccttgggggttgcaggctgcccccttcctgccagaccggaggggctggggggatcccagcagggggagggcaatcccttcaccccagttgccaaacagaccccccaccccctggattttccttctccctccatcccttgacggttctggccttcccaaactgcttttgatcttttgattcctcttgggctgaagcagaccaagttccccccaggcaccccagttgtgggggagcctgtattttttttaacaacatccccattccccacctggtcctcccccttcccatgctgccaacttctaaccgcaatagtg

SEQ ID NO: 66 - RNA, 128 nt, synthetic construct
  source 1..128: mol_type = other RNA; note; note (original language) = B9 mRNA sequence (COX4I1 3'UTR)
gagatgctggcctgcgcctgcacctgcgcctggctctgtcaccgccatgcaactccatgcctatttactggaaacctgttatgccaaacagttgtaccactgctaataaatgaccagtttacctgaaa

SEQ ID NO: 67 - RNA, 319 nt, synthetic construct
  source 1..319: mol_type = other RNA; note; note (original language) = B10 mRNA sequence (COX4I1 3'UTR)
agggacccacaggcgcgcccagcagctctcggaagcgttgtatcgcattaagttcaaggagagctttgctgagatgaacaggggctcgaacgagtggaagacggttgtgggcggtgccatgttcttcatcggtttcaccgcgctcgttatcatgtggcagaagcactatgggcttagcctccaagtgggactacgaaaagaacgagtggaagaagtgagagatgctggcctgcgcctgcacctgcgcctggctctgtcaccgccatgcaactccatgcctatttactggaaacctgttatgccaaacagttgtaccact

SEQ ID NO: 68 - RNA, 303 nt, synthetic construct
  source 1..303: mol_type = other RNA; note; note (original language) = B11 mRNA sequence (COX4I1 3'UTR)
agaggaccttctgcttttagcttattttgttgctaactttttacaaacaaagggctaattttaaaatgtcagtgttgtcagtggtcagaaaccgtgtgtttgagcgggtgttgagtggcaggtggctctgctgacctggtggctggtgtgtcgggaggatttaacctgtgtgagggattggcctagaaacaacctgttgagatagtcttgccccataacctgtctcacaccgtagtgtacggccccctcccgcaaagctttgacaaagagtgggtggccaagcagaccaagaggatgctggac

SEQ ID NO: 69 - RNA, 232 nt, synthetic construct
  source 1..232: mol_type = other RNA; note; note (original language) = B12 mRNA sequence (CTSB 3'UTR)
tctgccgtgggcctgtcgtgccagtcctgggggcgagatcgggagaatcacgtcctggaactgcatgttcttgcgactcttgggacttcatcttaacttctcgctgccccagccatgttttcaaccatggcatccctcccccaattagttccctgtcatcctcgtcaaccttctctgtaagtgcctggtaagcttgcccttgcttaagaactcaaaacatagctgtgctcta

SEQ ID NO: 70 - RNA, 115 nt, synthetic construct
  source 1..115: mol_type = other RNA; note; note (original language) = B13 mRNA sequence (FAM166A 3'UTR)
aaatgctttaatggtggtgtctgtacagcatggatgtggacagggaaaacagcaagtgcacacagtgggacaggccacaggacaggctgggagtgaataaagagttcacactgct

SEQ ID NO: 71 - RNA, 196 nt, synthetic construct
  source 1..196: mol_type = other RNA; note; note (original language) = B14 mRNA sequence (NDUFB9 3'UTR)
tatctaagtgtatcaatttaacatttataatcaccttacaagtaagttaaagtgcattccctggtcgttttggctttgtctttgattttgcttcagatctccttctctttagtcctttgtctgacttttttgccttcttgctatactttccctcaacctgcctctccactattttcttaggcatttttcagtcatg

SEQ ID NO: 72 - RNA, 54 nt, synthetic construct
  source 1..54: mol_type = other RNA; note; note (original language) = A1 mRNA sequence (ACTG1 5'UTR)
ctctcgcactctgttcttccgccgctccgccgtcgcgtttctctgccggtcgca

SEQ ID NO: 73 - RNA, 185 nt, synthetic construct
  source 1..185: mol_type = other RNA; note; note (original language) = A2 mRNA sequence (ATP6V0B 5'UTR)
gggcgggcggacagactgcgggacggacggtggacgctgggacgcgtttgtagctccggccccgccgttccgacccccgccgccgtcgccgccatgacggggctagcactgctctactccggggtcttcgtggccttctgggcctgcgcgctggccgtgggttcctgacggagacttcgcccttc

SEQ ID NO: 74 - RNA, 81 nt, synthetic construct
  source 1..81: mol_type = other RNA; note; note (original language) = A3 mRNA sequence (ATP6V0B 5'UTR)
agactgcgggacggacggtggacgctgggacgcgtttgtagctccggccccgccgttccgacccccgccgccgtcgccgcc

SEQ ID NO: 75 - RNA, 30 nt, synthetic construct
  source 1..30: mol_type = other RNA; note; note (original language) = A4 mRNA sequence (ATP6V0E1 5'UTR)
ggggtaggggttggcgctcaggcggcgacc

SEQ ID NO: 76 - RNA, 80 nt, synthetic construct
  source 1..80: mol_type = other RNA; note; note (original language) = A5 mRNA sequence (ATP6V0E1 5'UTR)
gtcacgcggtcagctattgacacttcctggtgggatccgagtgaggcgacggggtaggggttggcgctcaggcggcgacc

SEQ ID NO: 77 - RNA, 234 nt, synthetic construct
  source 1..234: mol_type = other RNA; note; note (original language) = A6 mRNA sequence (CFL1 5'UTR)
ggccggcgggaagactccgttacccagcgagcgaggcggcggcgcagggccagcggactccatttcccgtcggctcgcggtgggagcgccggaagcccgccccacccctcattgtgcggctcctactaaacggaaggggccgggagaggccgcgttcagtcgggtcccggcagcggctgcagcgctctcgtcttctgcggctctcggtgccctctccttttcgtttccggaaac

SEQ ID NO: 78 - RNA, 128 nt, synthetic construct
  source 1..128: mol_type = other RNA; note; note (original language) = A7 mRNA sequence (CFL1 5'UTR)
ctcctggctcgggcaccccgaagcacgacgcagagtaggaagagtttaaagacctcgaggcctctgggcacttgagtttggcctccggtgtggctgtctctgatggtgtcatcaaggtgttcaacgac

SEQ ID NO: 79 - RNA, 151 nt, synthetic construct
  source 1..151: mol_type = other RNA; note; note (original language) = A8 mRNA sequence (CFL1 5'UTR)
acgtggccggcttcttctgcagttccggggagtttgggggaccagatttaccttggattgcccctccctctcctggctcgggcaccccgaagcacgacgcagagcctccggtgtggctgtctctgatggtgtcatcaaggtgttcaacgac

SEQ ID NO: 80 - RNA, 70 nt, synthetic construct
  source 1..70: mol_type = other RNA; note; note (original language) = A9 mRNA sequence (COX4I1 5'UTR)
gcggccttgctctcttccggtcgcgggacaccgggtgtagagggcggtcgcggcgggcagtggcggcaga

SEQ ID NO: 81 - RNA, 46 nt, synthetic construct
  source 1..46: mol_type = other RNA; note; note (original language) = A10 mRNA sequence (COX4I1 5'UTR)
gggacaccgggtgtagagggcggtcgcggcgggcagtggcggcaga

SEQ ID NO: 82 - RNA, 71 nt, synthetic construct
  source 1..71: mol_type = other RNA; note; note (original language) = A11 mRNA sequence (COX4I1 5'UTR)
cgcggccttgctctcttccggtcgcgggacaccgggtgtagagggcggtcgcggcgggcagtggcggcaga

SEQ ID NO: 83 - RNA, 137 nt, synthetic construct
  source 1..137: mol_type = other RNA; note; note (original language) = A12 mRNA sequence (CUSB 5'UTR)
ggccggggctggcccaggctacggcggctgcagggctccggcaaccgctccggcaacgccaaccgctccgctgcgcgcaggctgggctgcaggctctcggctgcagcgctgggtggatctaggatccggcttccaac

SEQ ID NO: 84 - RNA, 55 nt, synthetic construct
  source 1..55: mol_type = other RNA; note; note (original language) = A13 mRNA sequence (FAM166A 5'UTR)
aagggagctggatgccgggagggactggagccagcaaggccagagtgaaagcaaa

SEQ ID NO: 85 - RNA, 56 nt, synthetic construct
  source 1..56: mol_type = other RNA; note; note (original language) = A14 mRNA sequence (NDUFB9 5'UTR)
gcagcaggcgtgcagtttcccggctctccgcgcggccggggaaggtcagcgccgta

SEQ ID NO: 86 - RNA, 68 nt, synthetic construct
  source 1..68: mol_type = other RNA; note; note (original language) = A15 mRNA sequence (CHCHD10 5'UTR)
ggcatttgtccccgcgacagcaccgctgccgccgtctctaaggtcgcccgggtcccaccgccgccacc

SEQ ID NO: 87 - RNA, 46 nt, synthetic construct
  source 1..46: mol_type = other RNA; note; note (original language) = A16 mRNA sequence (CHCHD10 5'UTR)
ccgctgccgccgtctctaaggtcgcccgggtcccaccgccgccacc

SEQ ID NO: 88 - RNA, 41 nt, synthetic construct
  source 1..41: mol_type = other RNA; note; note (original language) = A17 mRNA sequence (SLC38A2 5'UTR)
atgtcttttttgtgtgtttgttttcatggtattcctatgaa

SEQ ID NO: 89 - RNA, 48 nt, synthetic construct
  source 1..48: mol_type = other RNA; note; note (original language) = A18 mRNA sequence (NDUFA11 5'UTR)
gcttcccgagctggcggggtccgtggtgcgggatcgagattgcgggct

SEQ ID NO: 90 - RNA, 69 nt, synthetic construct
  source 1..69: mol_type = other RNA; note; note (original language) = A19 mRNA sequence (NDUFV3 5'UTR)
ggcggctgttcaggcgcgggtgcgcgcgcagctgctgtggccctgcttggtgcgcccgctgtcaccgcc

SEQ ID NO: 91 - RNA, 128 nt, synthetic construct
  source 1..128: mol_type = other RNA; note; note (original language) = A20 mRNA sequence (PRDX5 5'UTR)
cgcgcctgcgcagtggaggcggcccaggcccgccttccgcagggtgtcgccgctgtgccgctagcggtgccccgcctgctgcggtggcaccagccaggaggcggagtggaagtggccgtggggcgggt

SEQ ID NO: 92 - RNA, 59 nt, synthetic construct
  source 1..59: mol_type = other RNA; note; note (original language) = A21 mRNA sequence (GUK1 5'UTR)
cagcagatggggactagaggccgcactgctatccacagcctctcttctcacccccaggc

SEQ ID NO: 93 - RNA, 68 nt, synthetic construct
  source 1..68: mol_type = other RNA; note; note (original language) = A22 mRNA sequence (GUK1 5'UTR)
gctggccgggctggctgcggccgccctgggccgggccccaccggacgcctctcttctcacccccaggc

SEQ ID NO: 94 - RNA, 96 nt, synthetic construct
  source 1..96: mol_type = other RNA; note; note (original language) = A23 mRNA sequence (GUK1 5'UTR)
agaggtggccccggatgctgcggcgcccgctggccgggctggctgcggccgccctgggccgggccccaccggacgcctctcttctcacccccaggc

SEQ ID NO: 95 - RNA, 37 nt, synthetic construct
  source 1..37: mol_type = other RNA; note; note (original language) = A24 mRNA sequence (IAH1 5'UTR)
tggctggcggccccgccccgccccgcccggctgctcc

SEQ ID NO: 96 - RNA, 59 nt, synthetic construct
  source 1..59: mol_type = other RNA; note; note (original language) = A25 mRNA sequence (ABHD16A 5'UTR)
ggagggcggggccggcagggggacctgctgctggaagagcagcggcccgagccggggcc

SEQ ID NO: 97 - RNA, 132 nt, synthetic construct
  source 1..132: mol_type = other RNA; note; note (original language) = A26 mRNA sequence (SLC25A39 5'UTR)
tttcggcgtcggcctaggtgcgctgcgagcgcgcgcggaccgcgcacaggcggcggagccggtatgggcccgcctgaccctgggcgccgcgccgcacgagcaccagcctagagccaggactgaagcttcaag

SEQ ID NO: 98 - RNA, 51 nt, synthetic construct
  source 1..51: mol_type = other RNA; note; note (original language) = A27 mRNA sequence (AUPIF1 5'UTR)
cgagagactgcttgctgcggcagagacgccagaggtgcagctccagcagca

SEQ ID NO: 99 - RNA, 71 nt, synthetic construct
  source 1..71: mol_type = other RNA; note; note (original language) = A28 mRNA sequence (ANAPC11 5'UTR)
cggagtttcgtcatgttggccaggcccatttgagatctttgaagatatcctcaacgtgaggctctgctgcc

SEQ ID NO: 100 - RNA, 55 nt, synthetic construct
  source 1..55: mol_type = other RNA; note; note (original language) = A29 mRNA sequence (ANAPC11 5'UTR)
gggcgcggcttcggcgggcggcagccgctgcagacgagctgcgggctctgctgcc

SEQ ID NO: 101 - RNA, 48 nt, synthetic construct
  source 1..48: mol_type = other RNA; note; note (original language) = A30 mRNA sequence (CCDC12 5'UTR)
gcctgcgcgatgcaagacgggagaaaaggaggggcgtacgcgggcaag

SEQ ID NO: 102 - RNA, 132 nt, synthetic construct
  source 1..132: mol_type = other RNA; note; note (original language) = A31 mRNA sequence (MRPL14 5'UTR)
atcgcgtccgccgggctgggcctggcgcgcaggcgctaggaagaggccgcgtggggcgaaggcggcgcttggctggtggggcccgcggcgggattttcccgggcggcgagagcggatctatcttgggatccc

SEQ ID NO: 103 - RNA, 27 nt, synthetic construct
  source 1..27: mol_type = other RNA; note; note (original language) = A32 mRNA sequence (APOA1BP 5'UTR)
gccgggggcgcgcgctctgcgagctgg

SEQ ID NO: 104 - RNA, 43 nt, synthetic construct
  source 1..43: mol_type = other RNA; note; note (original language) = A33 mRNA sequence (APOA1BP 5'UTR)
gccggggccgggccgggccgggggcgcgcgctctgcgagctgg

SEQ ID NO: 105 - RNA, 47 nt, synthetic construct
  source 1..47: mol_type = other RNA; note; note (original language) = Mod. 5'UTR mRNA sequence
gggaaataagagagaaaagaagagtaagaagaaatataagagccacc

SEQ ID NO: 106 - RNA, 119 nt, synthetic construct
  source 1..119: mol_type = other RNA; note; note (original language) = a-globin 3'UTR mRNA sequence
tgataataggctggagcctcggtggccatgcttcttgccccttgggcctccccccagcccctcctccccttcctgcacccgtacccccgtggtctttgaataaagtctgagtgggcggc

SEQ ID NO: 107 - RNA, 52 nt, synthetic construct; identical to SEQ ID NO: 50
  source 1..52: mol_type = other RNA; note; note (original language) = a-1 globin 5'UTR mRNA sequence

SEQ ID NO: 108 - RNA, 317 nt, synthetic construct
  source 1..317: mol_type = other RNA; note; note (original language) = haplogroup U8b1b1 mitochondrion 3'UTR mRNA sequence
ctcgagctggtactgcatgcacgcaatgctagctgcccctttcccgtcctgggtaccccgagtctcccccgacctcgggtcccaggtatgctcccacctccacctgccccactcaccacctctgctagttccagacacctgctatactaatcgctagccgcgtcgctccccagggttggtcaatttcgtgccagccacaccgagacctggtccagagcccaagcacgccacacccccacgggaaacagcagtgattaacctttagcaataaacgaaagtttaactaacagcaatgcagctcaaaacgcttagcctag

SEQ ID NO: 109 - protein, 728 aa, Homo sapiens
  source 1..728: note; note (original language) = Amino acid sequence of hHGF
MWVTKLLPALLLQHVLLHLLLLPIAIPYAEGQRKRRNTIHEFKKSAKTTLIKIDPALKIKTKKVNTADQCANRCTRNKGLPFTCKAFVFDKARKQCLWFPFNSMSSGVKKEFGHEFDLYENKDYIRNCIIGKGRSYKGTVSITKSGIKCQPWSSMIPHEHSFLPSSYRGKDLQENYCRNPRGEEGGPWCFTSNPEVRYEVCDIPQCSEVECMTCNGESYRGLMDHTESGKICQRWDHQTPHRHKFLPERYPDKGFDDNYCRNPDGQPRPWCYTLDPHTRWEYCAIKTCADNTMNDTDVPLETTECIQGQGEGYRGTVNTIWNGIPCQRWDSQYPHEHDMTPENFKCKDLRENYCRNPDGSESPWCFTTDPNIRVGYCSQIPNCDMSHGQDCYRGNGKNYMGNLSQTRSGLTCSMWDKNMEDLHRHIFWEPDASKLNENYCRNPDDDAHGPWCYTGNPLIPWDYCPISRCEGDTTPTIVNLDHPVISCAKTKQLRVVNGIPTRTNIGWMVSLRYRNKHICGGSLIKESWVLTARQCFPSRDLKDYEAWLGIHDVHGRGDEKCKQVLNVSQLVYGPEGSDLVLMKLARPAVLDDFVSTIDLPNYGCTIPEKTSCSVYGWGYTGLINYDGLLRVAHLYIMGNEKCSQHHRGKVTLNESEICAGAEKIGSGPCEGDYGGPLVCEQHKMRMVLGVIVPGRGCAIPNRPGIFVRVAYYAKWIHKIILTYKVPQS

SEQ ID NO: 110 - DNA, 2187 bp, synthetic construct
  source 1..2187: mol_type = other DNA; note; note (original language) = Nucleotide sequence of hHGF
atgtgggtgaccaaactcctgccagccctgctgctgcagcatgtcctcctgcatctcctcctgctccccatcgccatcccctatgcagagggacaaaggaaaagaagaaatacaattcatgaattcaaaaaatcagcaaagactaccctaatcaaaatagatccagcactgaagataaaaaccaaaaaagtgaatactgcagaccaatgtgctaatagatgtactaggaataaaggacttccattcacttgcaaggcttttgtttttgataaagcaagaaaacaatgcctctggttccccttcaatagcatgtcaagtggagtgaaaaaagaatttggccatgaatttgacctctatgaaaacaaagactacattagaaactgcatcattggtaaaggacgcagctacaagggaacagtatctatcactaagagtggcatcaaatgtcagccctggagttccatgataccacacgaacacagctttttgccttcgagctatcggggtaaagacctacaggaaaactactgtcgaaatcctcgaggggaagaagggggaccctggtgtttcacaagcaatccagaggtacgctacgaagtctgtgacattcctcagtgttcagaagttgaatgcatgacctgcaatggggagagttatcgaggtctcatggatcatacagaatcaggcaagatttgtcagcgctgggatcatcagacaccacaccggcacaaattcttgcctgaaagatatcccgacaagggctttgatgataattattgccgcaatcccgatggccagccgaggccatggtgctatactcttgaccctcacacccgctgggagtactgtgcaattaaaacatgcgctgacaatactatgaatgacactgatgttcctttggaaacaactgaatgcatccaaggtcaaggagaaggctacaggggcactgtcaataccatttggaatggaattccatgtcagcgttgggattctcagtatcctcacgagcatgacatgactcctgaaaatttcaagtgcaaggacctacgagaaaattactgccgaaatccagatgggtctgaatcaccctggtgttttaccactgatccaaacatccgagttggctactgctcccaaattccaaactgtgatatgtcacatggacaagattgttatcgtgggaatggcaaaaattatatgggcaacttatcccaaacaagatctggactaacatgttcaatgtgggacaagaacatggaagacttacatcgtcatatcttctgggaaccagatgcaagtaagctgaatgagaattactgccgaaatccagatgatgatgctcatggaccctggtgctacacgggaaatccactcattccttgggattattgccctatttctcgttgtgaaggtgataccacacctacaatagtcaatttagaccatcccgtaatatcttgtgccaaaacgaaacaattgcgagttgtaaatgggattccaacacgaacaaacataggatggatggttagtttgagatacagaaataaacatatctgcggaggatcattgataaaggagagttgggttcttactgcacgacagtgtttcccttctcgagacttgaaagattatgaagcttggcttggaattcatgatgtccacggaagaggagatgagaaatgcaaacaggttctcaatgtttcccagctggtatatggccctgaaggatcagatctggttttaatgaagcttgccaggcctgctgtcctggatgattttgttagtacgattgatttacctaattatggatgcacaattcctgaaaagaccagttgcagtgtttatggctggggctacactggattgatcaactatgatggcctattacgagtggcacatctctatataatgggaaatgagaaatgcagccagcatcatcgagggaaggtgactctgaatgagtctgaaatatgtgctggggctgaaaagattggatcaggaccatgtgagggggattatggtggcccacttgtttgtgagcaacataaaatgagaatggttcttggtgtcattgttcctggtcgtggatgtgccattccaaatcgtcctggtatttttgtccgagtagcatattatgcaaaatggatacacaaaattattttaacatataaggtaccacagtcatag

SEQ ID NO: 111 - DNA, 2187 bp, synthetic construct
  source 1..2187: mol_type = other DNA; note; note (original language) = hHGF codon-optimized sequence 1 (hHGF-OS1)
atgtgggtgaccaaactgctccccgctctgctgctgcagcatgtgctgctccacctgctgctgctgccaatcgccatcccctacgctgaaggacagcggaagcgcagaaacacaattcacgaattcaagaagtccgccaaaacaacactgatcaagatcgaccctgccctgaaaatcaaaaccaagaaggtgaacactgccgatcagtgcgccaacagatgcacaagaaacaaaggcctgcccttcacatgcaaggcctttgtgttcgacaaggccagaaagcagtgcctgtggttccctttcaacagcatgagctctggcgtgaagaaagagttcggccacgaattcgacctgtacgagaacaaggattacatcagaaattgtatcatcggcaagggcagaagctacaaaggcacagtgtccatcaccaaaagcggcattaagtgtcagccttggagcagcatgatccctcacgagcacagcttcctgcctagctcttacagaggcaaggacctgcaggagaattactgccggaaccctagaggcgaggaaggcggcccttggtgctttaccagcaaccctgaggtgcggtacgaggtgtgtgacatcccccagtgcagcgaagtggaatgcatgacctgtaatggcgagagctacagaggcctcatggaccatacagagagcggaaagatttgtcaaagatgggatcaccagacacctcacagacacaaattcctgcccgaaagatatcctgacaagggcttcgacgacaactactgcagaaatcctgatggccaacccagaccttggtgctacaccctggatcctcataccagatgggagtactgtgccatcaagacctgcgctgataataccatgaacgacaccgatgtgcctctggaaacaaccgagtgcatccagggacagggcgaaggctaccggggcaccgtgaacaccatctggaacggcatcccctgccagagatgggacagccagtacccccacgaacacgatatgacccctgagaacttcaagtgcaaggacctgagagaaaattactgcagaaacccagacggaagcgagtctccttggtgttttaccaccgaccccaacatccgggtgggttactgcagccaaatccccaattgcgacatgagccacggccaggactgctaccggggaaacggcaaaaactacatgggcaatctgagccagacccggagcggtctgacctgctccatgtgggataagaacatggaagatctgcaccggcacatcttctgggagcctgacgcttctaagctgaacgagaactactgtaggaacccagacgacgatgcccacggtccctggtgctacaccggcaacccgctgatcccttgggactattgtcctatcagccgctgcgagggcgatacaacacctaccatcgtgaacctggaccaccctgtgatctcttgcgccaagaccaagcagctgagagtggtgaacggcatcccaacacggaccaacatcggatggatggtctccctgagataccggaacaagcacatctgcggcggctctctgatcaaggaatcttgggtcctgaccgccagacagtgcttccccagccgggacctgaaggactatgaggcctggctgggaatccacgacgtgcacggcagaggcgacgagaagtgcaagcaagtgctgaacgtgtcccagctggtgtacggccctgagggatctgatctggtcctgatgaaactggccagacccgccgtgctggacgactttgtgtccaccatcgacctgcctaactacggctgcaccatccctgaaaagaccagctgcagcgtgtacggctggggctatacaggcctgatcaactacgacggtctgctgcgggttgctcacctgtacatcatgggcaacgagaagtgcagccagcaccacagaggaaaggttacacttaacgagagcgagatctgcgccggcgccgagaaaatcggctccggcccttgtgaaggcgactacggaggccctctggtgtgcgaacagcacaagatgagaatggtgctgggcgtgatcgtgcccggaagaggctgtgcaatccctaataggcccggcattttcgtgcgggtggcctactacgccaagtggatccacaagatcatcctgacgtacaaggtgcctcagagctga

SEQ ID NO: 112 - DNA, 2187 bp, synthetic construct
  source 1..2187: mol_type = other DNA; note; note (original language) = hHGF codon-optimized sequence 2 (hHGF-OS2)
atgtgggtcaccaaactgctgcccgccctgctgctgcagcacgtgctcctgcacctgctgctgctgcctatcgccatcccttacgccgaaggccagagaaagcggagaaataccattcacgaatttaagaagagcgccaagaccacactgatcaagatcgaccctgccctgaaaatcaagaccaagaaagtgaacacagccgaccaatgcgctaatagatgcacaagaaacaaaggcctgcctttcacctgcaaggccttcgtgttcgataaggccagaaagcagtgcctgtggttccccttcaacagcatgagcagcggcgtgaagaaagaattcggtcacgagttcgacctgtacgagaataaggactacattagaaactgcatcatcggcaagggccggagctacaagggcaccgtgagcatcaccaagtctggcatcaagtgccagccatggagttccatgatccctcatgagcacagcttcctgccaagctcttaccggggaaaggatctgcaggagaactattgtagaaatcccagaggcgaggaaggaggaccctggtgttttaccagcaacccagaggtgcggtacgaggtgtgcgacataccccagtgcagcgaggtggaatgcatgacatgcaacggcgagagctaccggggcctgatggaccacacagagagcggcaaaatctgccaaagatgggatcaccagacccctcataggcacaagttcctgcccgagagataccctgacaagggcttcgacgacaattactgccggaaccctgatggacagcctagaccttggtgctacaccctggaccctcacaccagatgggaatactgcgccatcaagacatgtgccgataacaccatgaacgacaccgatgtgccactcgagacaactgagtgtatccagggccagggcgagggctacaggggcaccgtgaacaccatctggaacggcatcccttgtcagcggtgggacagccaatacccccacgaacatgatatgaccccagaaaacttcaagtgcaaagatctgcgggaaaactactgtagaaaccctgacggctccgagagcccttggtgcttcaccaccgaccctaacatcagggtgggctactgtagccagatccccaactgcgacatgagccacggtcaggactgctacagaggaaacggcaagaattacatgggcaacctgagccagaccagaagcggcctgacctgcagcatgtgggacaaaaacatggaagatctgcaccggcacatcttttgggagcctgacgccagcaagctgaatgagaactactgtcggaaccctgacgacgatgctcacggcccttggtgctacacaggcaaccctctgatcccttgggactattgtcctattagcaggtgtgaaggcgacacgacccctacaatcgtgaacctggatcacccagtgatcagctgtgctaaaacaaagcaactgagagtggtgaatggtatcccgacccggaccaacatcggatggatggtcagcctgcggtacagaaacaagcacatctgcggcggtagcctgatcaaggaatcctgggtgttgacagccagacagtgttttcccagcagagatctgaaggactacgaggcctggctgggcatccacgacgtgcacggcagaggcgacgagaagtgcaagcaggttctgaacgtgtcccagctggtgtacggccccgagggctctgatctggttctgatgaagcttgctagacccgctgtgctggatgacttcgtgtccaccatcgacctgccaaattacggatgtacaattcctgaaaagacctcctgttctgtgtacggctggggctacaccggactcatcaactatgacggcctgctgagagtggcccacctgtatatcatgggcaacgagaagtgcagccagcaccatagaggcaaggtgaccctgaacgagtctgaaatctgcgccggagccgagaaaatcggatctggcccctgcgaaggagattacggcggccctctggtctgcgagcagcacaagatgagaatggtgctgggcgtgatcgtgcccggcagaggctgcgccatccctaaccggcctggaatcttcgtgcgcgtggcctattacgccaaatggatccacaaaatcatcctgacatacaaggtcccacagtcttga

SEQ ID NO: 113 - DNA, 2187 bp, synthetic construct
  source 1..2187: mol_type = other DNA; note; note (original language) = hHGF codon-optimized sequence 3 (hHGF-OS3)
atgtgggtgaccaagctgctgcccgccctgctcctgcagcacgtgctgctgcacctgctcctgctgcccatcgccatcccctacgccgaggggcagagaaagagaagaaacaccatccacgagttcaagaagagcgccaagaccaccctgatcaagatcgaccccgccctgaagatcaagaccaagaaggtgaacaccgccgatcagtgcgccaacagatgcacaagaaacaagggcctgcccttcacctgcaaggccttcgtgttcgacaaggctagaaagcagtgcctgtggttccccttcaacagcatgagcagcggcgtgaagaaggagttcggccacgagttcgacctgtacgagaacaaggactacatcagaaactgcatcatcggcaagggcagaagctacaagggcaccgtgagcatcaccaagagcggcatcaagtgtcagccctggagcagcatgatcccccatgagcacagcttcctgcctagcagctacagagggaaggacctgcaagagaactactgcagaaaccctagaggcgaggagggcggcccttggtgtttcacaagcaatcccgaggtgagatacgaggtgtgcgacatccctcagtgcagcgaggtggagtgcatgacctgcaacggcgaaagctatagaggcctgatggaccacaccgagagcggcaagatttgtcagcggtgggatcaccaaaccccccacagacacaagttcctgcccgagagataccccgacaagggcttcgacgacaattactgtagaaaccccgacgggcagcctagaccctggtgttacaccctggacccccacacaagatgggagtactgcgccatcaagacctgcgccgacaacaccatgaacgacaccgacgtgcccctggagaccaccgagtgcatccaaggccaaggcgagggctacagaggcaccgtgaacaccatctggaacggcattccctgtcagagatgggacagccaatacccccatgaacacgatatgacccccgagaacttcaagtgcaaggacctgagagagaactactgccggaaccccgatggcagcgaatccccttggtgcttcaccaccgaccccaacatcagagtgggctactgcagccaaatccccaactgcgacatgagccacggccaagactgttacagagggaacggcaagaactacatgggcaacctgagccaaacaagaagcggcctgacctgcagcatgtgggacaagaacatggaggacctgcacagacacatcttctgggagcccgacgctagcaagctgaacgagaactactgtcggaaccccgacgacgatgcccacggcccctggtgctacaccggcaaccccctgatcccctgggactactgccccatcagcagatgcgagggcgacaccacccccaccatcgtgaacctggaccaccccgtgatcagctgtgccaagaccaagcaactgagagtggtgaacggcatccccacaagaaccaacattggctggatggtgagcctgagatacagaaacaagcacatctgcggcggcagcctgatcaaggagagctgggtgctgaccgctagacagtgcttccctagcagagacctgaaggactacgaggcctggctgggcatccacgacgtgcacggcagaggcgacgagaagtgtaaacaagtgctgaacgtgagccaactggtgtacggccccgagggcagcgacctggtgctgatgaagctggctagacccgccgtgctggacgacttcgtgagcaccatcgacctgcccaactacggctgcaccatccccgagaagacaagctgcagcgtgtacggctggggctacaccggcctgatcaactacgacggcctgctgagagtggcccacctgtacatcatgggcaacgagaagtgcagccaacaccaccggggcaaagtgaccctgaacgagagcgagatctgcgccggggctgagaaaatcggcagcggcccctgcgagggggactacgggggccccctggtgtgcgagcagcacaagatgagaatggtgctgggcgtgatcgtgcccggcagaggctgcgccatccccaacagacccggcatcttcgtgagagtggcctactacgccaagtggatccacaagatcatcctgacctacaaggtgcctcagagctga

SEQ ID NO: 114 - DNA, 2512 bp, synthetic construct
  source 1..2512: mol_type = other DNA; note; note (original language) = 5'UTR-hHGF-α globin 3'UTR-A30L70 (Mod.-hHGF-OS2)
gggaaataagagagaaaagaagagtaagaagaaatataagagccaccgctagccttaaggccaccatgtgggtcaccaaactgctgcccgccctgctgctgcagcacgtgctcctgcacctgctgctgctgcctatcgccatcccttacgccgaaggccagagaaagcggagaaataccattcacgaatttaagaagagcgccaagaccacactgatcaagatcgaccctgccctgaaaatcaagaccaagaaagtgaacacagccgaccaatgcgctaatagatgcacaagaaacaaaggcctgcctttcacctgcaaggccttcgtgttcgataaggccagaaagcagtgcctgtggttccccttcaacagcatgagcagcggcgtgaagaaagaattcggtcacgagttcgacctgtacgagaataaggactacattagaaactgcatcatcggcaagggccggagctacaagggcaccgtgagcatcaccaagtctggcatcaagtgccagccatggagttccatgatccctcatgagcacagcttcctgccaagctcttaccggggaaaggatctgcaggagaactattgtagaaatcccagaggcgaggaaggaggaccctggtgttttaccagcaacccagaggtgcggtacgaggtgtgcgacataccccagtgcagcgaggtggaatgcatgacatgcaacggcgagagctaccggggcctgatggaccacacagagagcggcaaaatctgccaaagatgggatcaccagacccctcataggcacaagttcctgcccgagagataccctgacaagggcttcgacgacaattactgccggaaccctgatggacagcctagaccttggtgctacaccctggaccctcacaccagatgggaatactgcgccatcaagacatgtgccgataacaccatgaacgacaccgatgtgccactcgagacaactgagtgtatccagggccagggcgagggctacaggggcaccgtgaacaccatctggaacggcatcccttgtcagcggtgggacagccaatacccccacgaacatgatatgaccccagaaaacttcaagtgcaaagatctgcgggaaaactactgtagaaaccctgacggctccgagagcccttggtgcttcaccaccgaccctaacatcagggtgggctactgtagccagatccccaactgcgacatgagccacggtcaggactgctacagaggaaacggcaagaattacatgggcaacctgagccagaccagaagcggcctgacctgcagcatgtgggacaaaaacatggaagatctgcaccggcacatcttttgggagcctgacgccagcaagctgaatgagaactactgtcggaaccctgacgacgatgctcacggcccttggtgctacacaggcaaccctctgatcccttgggactattgtcctattagcaggtgtgaaggcgacacgacccctacaatcgtgaacctggatcacccagtgatcagctgtgctaaaacaaagcaactgagagtggtgaatggtatcccgacccggaccaacatcggatggatggtcagcctgcggtacagaaacaagcacatctgcggcggtagcctgatcaaggaatcctgggtgttgacagccagacagtgttttcccagcagagatctgaaggactacgaggcctggctgggcatccacgacgtgcacggcagaggcgacgagaagtgcaagcaggttctgaacgtgtcccagctggtgtacggccccgagggctctgatctggttctgatgaagcttgctagacccgctgtgctggatgacttcgtgtccaccatcgacctgccaaattacggatgtacaattcctgaaaagacctcctgttctgtgtacggctggggctacaccggactcatcaactatgacggcctgctgagagtggcccacctgtatatcatgggcaacgagaagtgcagccagcaccatagaggcaaggtgaccctgaacgagtctgaaatctgcgccggagccgagaaaatcggatctggcccctgcgaaggagattacggcggccctctggtctgcgagcagcacaagatgagaatggtgctgggcgtgatcgtgcccggcagaggctgcgccatccctaaccggcctggaatcttcgtgcgcgtggcctattacgccaaatggatccacaaaatcatcctgacatacaaggtcccacagtcttgataataggctggagcctcggtggccatgcttcttgccccttgggcctccccccagcccctcctccccttcctgcacccgtacccccgtggtctttgaataaagtctgagtgggcggcctcgagccgcggaaaaaaaaaaaaaaaaaaaaaaaaaaaaaagcatatgactaaaaaaaaaaaaaaaaaaaaaaaaaaaaaaaaaaaaaaaaaaaaaaaaaaaaaaaaaaaaaaaaaaaaaagtttaaacatttaaattctaga

SEQ ID NO: 115 - DNA, 2638 bp, synthetic construct
  source 1..2638: mol_type = other DNA; note; note (original language) = ACTG1 5'UTR-hHGF-CTSB 3'UTR-A30L70 (A1B12-hHGF-OS2)
ctctcgcactctgttcttccgccgctccgccgtcgcgtttctctgccggtcgcagctagcgccaccatgtgggtcaccaaactgctgcccgccctgctgctgcagcacgtgctcctgcacctgctgctgctgcctatcgccatcccttacgccgaaggccagagaaagcggagaaataccattcacgaatttaagaagagcgccaagaccacactgatcaagatcgaccctgccctgaaaatcaagaccaagaaagtgaacacagccgaccaatgcgctaatagatgcacaagaaacaaaggcctgcctttcacctgcaaggccttcgtgttcgataaggccagaaagcagtgcctgtggttccccttcaacagcatgagcagcggcgtgaagaaagaattcggtcacgagttcgacctgtacgagaataaggactacattagaaactgcatcatcggcaagggccggagctacaagggcaccgtgagcatcaccaagtctggcatcaagtgccagccatggagttccatgatccctcatgagcacagcttcctgccaagctcttaccggggaaaggatctgcaggagaactattgtagaaatcccagaggcgaggaaggaggaccctggtgttttaccagcaacccagaggtgcggtacgaggtgtgcgacataccccagtgcagcgaggtggaatgcatgacatgcaacggcgagagctaccggggcctgatggaccacacagagagcggcaaaatctgccaaagatgggatcaccagacccctcataggcacaagttcctgcccgagagataccctgacaagggcttcgacgacaattactgccggaaccctgatggacagcctagaccttggtgctacaccctggaccctcacaccagatgggaatactgcgccatcaagacatgtgccgataacaccatgaacgacaccgatgtgccactcgagacaactgagtgtatccagggccagggcgagggctacaggggcaccgtgaacaccatctggaacggcatcccttgtcagcggtgggacagccaatacccccacgaacatgatatgaccccagaaaacttcaagtgcaaagatctgcgggaaaactactgtagaaaccctgacggctccgagagcccttggtgcttcaccaccgaccctaacatcagggtgggctactgtagccagatccccaactgcgacatgagccacggtcaggactgctacagaggaaacggcaagaattacatgggcaacctgagccagaccagaagcggcctgacctgcagcatgtgggacaaaaacatggaagatctgcaccggcacatcttttgggagcctgacgccagcaagctgaatgagaactactgtcggaaccctgacgacgatgctcacggcccttggtgctacacaggcaaccctctgatcccttgggactattgtcctattagcaggtgtgaaggcgacacgacccctacaatcgtgaacctggatcacccagtgatcagctgtgctaaaacaaagcaactgagagtggtgaatggtatcccgacccggaccaacatcggatggatggtcagcctgcggtacagaaacaagcacatctgcggcggtagcctgatcaaggaatcctgggtgttgacagccagacagtgttttcccagcagagatctgaaggactacgaggcctggctgggcatccacgacgtgcacggcagaggcgacgagaagtgcaagcaggttctgaacgtgtcccagctggtgtacggccccgagggctctgatctggttctgatgaagcttgctagacccgctgtgctggatgacttcgtgtccaccatcgacctgccaaattacggatgtacaattcctgaaaagacctcctgttctgtgtacggctggggctacaccggactcatcaactatgacggcctgctgagagtggcccacctgtatatcatgggcaacgagaagtgcagccagcaccatagaggcaaggtgaccctgaacgagtctgaaatctgcgccggagccgagaaaatcggatctggcccctgcgaaggagattacggcggccctctggtctgcgagcagcacaagatgagaatggtgctgggcgtgatcgtgcccggcagaggctgcgccatccctaaccggcctggaatcttcgtgcgcgtggcctattacgccaaatggatccacaaaatcatcctgacatacaaggtcccacagtcttgataagggcccaccggttctgccgtgggcctgtcgtgccagtcctgggggcgagatcgggagaatcacgtcctggaactgcatgttcttgcgactcttgggacttcatcttaacttctcgctgccccagccatgttttcaaccatggcatccctcccccaattagttccctgtcatcctcgtcaaccttctctgtaagtgcctggtaagcttgcccttgcttaagaactcaaaacatagctgtgctctaccgcggaaaaaaaaaaaaaaaaaaaaaaaaaaaaaagcatatgactaaaaaaaaaaaaaaaaaaaaaaaaaaaaaaaaaaaaaaaaaaaaaaaaaaaaaaaaaaaaaaaaaaaaaagtttaaacatttaaattctaga

SEQ ID NO: 116 - DNA, 2652 bp, synthetic construct
  source 1..2652: mol_type = other DNA; note; note (original language) = CHCHD10 5'UTR-hHGF-CTSB 3'UTR-A30L70 (A15B12-hHGF-OS2)
ggcatttgtccccgcgacagcaccgctgccgccgtctctaaggtcgcccgggtcccaccgccgccaccgctagcgccaccatgtgggtcaccaaactgctgcccgccctgctgctgcagcacgtgctcctgcacctgctgctgctgcctatcgccatcccttacgccgaaggccagagaaagcggagaaataccattcacgaatttaagaagagcgccaagaccacactgatcaagatcgaccctgccctgaaaatcaagaccaagaaagtgaacacagccgaccaatgcgctaatagatgcacaagaaacaaaggcctgcctttcacctgcaaggccttcgtgttcgataaggccagaaagcagtgcctgtggttccccttcaacagcatgagcagcggcgtgaagaaagaattcggtcacgagttcgacctgtacgagaataaggactacattagaaactgcatcatcggcaagggccggagctacaagggcaccgtgagcatcaccaagtctggcatcaagtgccagccatggagttccatgatccctcatgagcacagcttcctgccaagctcttaccggggaaaggatctgcaggagaactattgtagaaatcccagaggcgaggaaggaggaccctggtgttttaccagcaacccagaggtgcggtacgaggtgtgcgacataccccagtgcagcgaggtggaatgcatgacatgcaacggcgagagctaccggggcctgatggaccacacagagagcggcaaaatctgccaaagatgggatcaccagacccctcataggcacaagttcctgcccgagagataccctgacaagggcttcgacgacaattactgccggaaccctgatggacagcctagaccttggtgctacaccctggaccctcacaccagatgggaatactgcgccatcaagacatgtgccgataacaccatgaacgacaccgatgtgccactcgagacaactgagtgtatccagggccagggcgagggctacaggggcaccgtgaacaccatctggaacggcatcccttgtcagcggtgggacagccaatacccccacgaacatgatatgaccccagaaaacttcaagtgcaaagatctgcgggaaaactactgtagaaaccctgacggctccgagagcccttggtgcttcaccaccgaccctaacatcagggtgggctactgtagccagatccccaactgcgacatgagccacggtcaggactgctacagaggaaacggcaagaattacatgggcaacctgagccagaccagaagcggcctgacctgcagcatgtgggacaaaaacatggaagatctgcaccggcacatcttttgggagcctgacgccagcaagctgaatgagaactactgtcggaaccctgacgacgatgctcacggcccttggtgctacacaggcaaccctctgatcccttgggactattgtcctattagcaggtgtgaaggcgacacgacccctacaatcgtgaacctggatcacccagtgatcagctgtgctaaaacaaagcaactgagagtggtgaatggtatcccgacccggaccaacatcggatggatggtcagcctgcggtacagaaacaagcacatctgcggcggtagcctgatcaaggaatcctgggtgttgacagccagacagtgttttcccagcagagatctgaaggactacgaggcctggctgggcatccacgacgtgcacggcagaggcgacgagaagtgcaagcaggttctgaacgtgtcccagctggtgtacggccccgagggctctgatctggttctgatgaagcttgctagacccgctgtgctggatgacttcgtgtccaccatcgacctgccaaattacggatgtacaattcctgaaaagacctcctgttctgtgtacggctggggctacaccggactcatcaactatgacggcctgctgagagtggcccacctgtatatcatgggcaacgagaagtgcagccagcaccatagaggcaaggtgaccctgaacgagtctgaaatctgcgccggagccgagaaaatcggatctggcccctgcgaaggagattacggcggccctctggtctgcgagcagcacaagatgagaatggtgctgggcgtgatcgtgcccggcagaggctgcgccatccctaaccggcctggaatcttcgtgcgcgtggcctattacgccaaatggatccacaaaatcatcctgacatacaaggtcccacagtcttgataagggcccaccggttctgccgtgggcctgtcgtgccagtcctgggggcgagatcgggagaatcacgtcctggaactgcatgttcttgcgactcttgggacttcatcttaacttctcgctgccccagccatgttttcaaccatggcatccctcccccaattagttccctgtcatcctcgtcaaccttctctgtaagtgcctggtaagcttgcccttgcttaagaactcaaaacatagctgtgctctaccgcggaaaaaaaaaaaaaaaaaaaaaaaaaaaaaagcatatgactaaaaaaaaaaaaaaaaaaaaaaaaaaaaaaaaaaaaaaaaaaaaaaaaaaaaaaaaaaaaaaaaaaaaaagtttaaacatttaaattctaga

SEQ ID NO: 117 - protein, 462 aa, Homo sapiens
  source 1..462: note; note (original language) = PD-1 antibody heavy chain amino acid sequence
MEWSWVFLFFLSVTTGVHSEVQLVESGGGLVQPGGSLRLSCAASGFTFSSYMMSWVRQAPGKGLEWVATISGGGANTYYPDSVKGRFTISRDNAKNSLYLQMNSLRAEDTAVYYCARQLYYFDYWGQGTTVTVSSASTKGPSVFPLAPCSRSTSESTAALGCLVKDYFPEPVTVSWNSGALTSGVHTFPAVLQSSGLYSLSSVVTVPSSSLGTKTYTCNVDHKPSNTKVDKRVESKYGPPCPPCPAPEFLGGPSVFLFPPKPKDTLMISRTPEVTCVVVDVSQEDPEVQFNWYVDGVEVHNAKTKPREEQFNSTYRVVSVLTVLHQDWLNGKEYKCKVSNKGLPSSIEKTISKAKGQPREPQVYTLPPSQEEMTKNQVSLTCLVKGFYPSDIAVEWESNGQPENNYKTTPPVLDSDGSFFLYSRLTVDKSRWQEGNVFSCSVMHEALHNHYTQKSLSLSLGK

SEQ ID NO: 118 - protein, 234 aa, Homo sapiens
  source 1..234: note; note (original language) = PD-1 antibody light chain amino acid sequence
MSVPTQVLGLLLLWLTDARCDIQMTQSPSSLSASVGDRVTITCLASQTIGTWLTWYQQKPGKAPKLLIYTATSLADGVPSRFSGSGSGTDFTLTISSLQPEDFATYYCQQVYSIPWTFGGGTKVEIKRTVAAPSVFIFPPSDEQLKSGTASVVCLLNNFYPREAKVQWKVDNALQSGNSQESVTEQDSKDSTYSLSSTLTLSKADYEKHKVYACEVTHQGLSSPVTKSFNRGEC

SEQ ID NO: 119 - DNA, 1386 bp, synthetic construct
  source 1..1386: mol_type = other DNA; note; note (original language) = PD-1 antibody heavy chain DNA sequence
atggaatggtcctgggtgttcctgttcttcctgtccgtgaccaccggcgtgcactccgaagtgcagctggtggaatctggcggcggactggtgcagcctggcggatctctgagactgtcttgtgccgcctccggcttcaccttctccagctacatgatgagctgggtgcgacaggcccctggcaagggactggaatgggtggccacaatctctggcggaggcgccaacacctactaccccgactctgtgaagggccggttcaccatctctcgggacaacgccaagaactccctgtacctgcagatgaacagcctgcgggccgaggacaccgccgtgtactactgtgcccggcagctgtactacttcgactactggggccagggcaccaccgtgaccgtgtcctctgcttctaccaagggcccctccgtgttccctctggctccttgctccagatccacctccgagtccaccgctgctctgggctgcctcgtgaaggactacttccccgagcctgtgacagtgtcctggaactctggcgccctgacctctggcgtgcacacctttccagcagtgctgcagtcctccggcctgtactccctgtcctccgtcgtgacagtgccctccagctctctgggcaccaagacctacacctgtaacgtggaccacaagccctccaacaccaaggtggacaagagagtggaatctaagtacggccctccctgccccccttgtcctgcccctgaatttctgggcggaccctctgtgtttctgttccccccaaagcccaaggacaccctgatgatctcccggacccccgaagtgacctgcgtggtggtggatgtgtcccaggaagatcccgaggtgcagttcaattggtacgtggacggcgtggaagtgcacaatgccaagaccaagcctagagaggaacagttcaactccacctaccgggtggtgtccgtgctgaccgtgctgcatcaggactggctgaacggcaaagagtacaagtgcaaggtgtccaacaagggcctgcccagctccatcgaaaagaccatctccaaggccaagggccagccccgggaaccccaggtgtacacactgcctccaagccaggaagagatgaccaagaaccaggtgtccctgacctgcctcgtgaaaggcttctacccctccgatatcgccgtggaatgggagtccaacggccagcctgagaacaactacaagaccaccccccctgtgctggactccgacggctccttctttctgtactctcgcctgaccgtggacaagtcccggtggcaggaaggcaacgtgttctcctgcagcgtgatgcacgaggccctgcacaaccactacacccagaagtccctgtccctgtctctgggaaag

SEQ ID NO: 120 - DNA, 702 bp, synthetic construct
  source 1..702: mol_type = other DNA; note; note (original language) = PD-1 antibody light chain DNA sequence
atgtccgtgcctacccaggtgctgggactgctgctgctgtggctgaccgacgccagatgcgacatccagatgacccagtccccctccagcctgtctgcctctgtgggcgacagagtgaccatcacctgtctggcctcccagaccatcggcacctggctgacctggtatcagcagaagcctggcaaggcccccaagctgctgatctacaccgccaccagtctggccgatggcgtgccctctagattctccggctctggctctggcaccgactttaccctgaccatcagctccctgcagcccgaggacttcgccacctactactgccagcaggtgtactccatcccctggacctttggcggaggcaccaaggtggaaatcaagcggaccgtggccgctccctccgtgttcatcttcccaccttccgacgagcagctgaagtccggaaccgccagtgtcgtgtgcctgctgaacaacttctacccccgcgaggccaaggtgcagtggaaggtggacaacgccctgcagtccggcaactcccaggaatccgtgaccgagcaggactccaaggacagcacctactccctgtcctccaccctgaccctgtccaaggccgactacgagaagcacaaggtgtacgcctgcgaagtgacccaccagggcctgtctagccccgtgaccaagtctttcaaccggggcgagtgc

SEQ ID NO: 121 - RNA, 1386 nt, synthetic construct
  source 1..1386: mol_type = other RNA; note; note (original language) = PD-1 antibody heavy chain mRNA sequence
atggaatggtcctgggtgttcctgttcttcctgtccgtgaccaccggcgtgcactccgaagtgcagctggtggaatctggcggcggactggtgcagcctggcggatctctgagactgtcttgtgccgcctccggcttcaccttctccagctacatgatgagctgggtgcgacaggcccctggcaagggactggaatgggtggccacaatctctggcggaggcgccaacacctactaccccgactctgtgaagggccggttcaccatctctcgggacaacgccaagaactccctgtacctgcagatgaacagcctgcgggccgaggacaccgccgtgtactactgtgcccggcagctgtactacttcgactactggggccagggcaccaccgtgaccgtgtcctctgcttctaccaagggcccctccgtgttccctctggctccttgctccagatccacctccgagtccaccgctgctctgggctgcctcgtgaaggactacttccccgagcctgtgacagtgtcctggaactctggcgccctgacctctggcgtgcacacctttccagcagtgctgcagtcctccggcctgtactccctgtcctccgtcgtgacagtgccctccagctctctgggcaccaagacctacacctgtaacgtggaccacaagccctccaacaccaaggtggacaagagagtggaatctaagtacggccctccctgccccccttgtcctgcccctgaatttctgggcggaccctctgtgtttctgttccccccaaagcccaaggacaccctgatgatctcccggacccccgaagtgacctgcgtggtggtggatgtgtcccaggaagatcccgaggtgcagttcaattggtacgtggacggcgtggaagtgcacaatgccaagaccaagcctagagaggaacagttcaactccacctaccgggtggtgtccgtgctgaccgtgctgcatcaggactggctgaacggcaaagagtacaagtgcaaggtgtccaacaagggcctgcccagctccatcgaaaagaccatctccaaggccaagggccagccccgggaaccccaggtgtacacactgcctccaagccaggaagagatgaccaagaaccaggtgtccctgacctgcctcgtgaaaggcttctacccctccgatatcgccgtggaatgggagtccaacggccagcctgagaacaactacaagaccaccccccctgtgctggactccgacggctccttctttctgtactctcgcctgaccgtggacaagtcccggtggcaggaaggcaacgtgttctcctgcagcgtgatgcacgaggccctgcacaaccactacacccagaagtccctgtccctgtctctgggaaag

SEQ ID NO: 122 - RNA, 702 nt, synthetic construct
  source 1..702: mol_type = other RNA; note; note (original language) = PD-1 antibody light chain mRNA sequence
atgtccgtgcctacccaggtgctgggactgctgctgctgtggctgaccgacgccagatgcgacatccagatgacccagtccccctccagcctgtctgcctctgtgggcgacagagtgaccatcacctgtctggcctcccagaccatcggcacctggctgacctggtatcagcagaagcctggcaaggcccccaagctgctgatctacaccgccaccagtctggccgatggcgtgccctctagattctccggctctggctctggcaccgactttaccctgaccatcagctccctgcagcccgaggacttcgccacctactactgccagcaggtgtactccatcccctggacctttggcggaggcaccaaggtggaaatcaagcggaccgtggccgctccctccgtgttcatcttcccaccttccgacgagcagctgaagtccggaaccgccagtgtcgtgtgcctgctgaacaacttctacccccgcgaggccaaggtgcagtggaaggtggacaacgccctgcagtccggcaactcccaggaatccgtgaccgagcaggactccaaggacagcacctactccctgtcctccaccctgaccctgtccaaggccgactacgagaagcacaaggtgtacgcctgcgaagtgacccaccagggcctgtctagccccgtgaccaagtctttcaaccggggcgagtgc

SEQ ID NO: 123 - DNA, 2478 bp, synthetic construct
  source 1..2478: mol_type = other DNA; note; note (original language) = 5'UTR-anti PD-1-a globin 3'UTR-A30L70 (Mod.-anti PD-1)
gggaaataagagagaaaagaagagtaagaagaaatataagagccaccatggaatggtcctgggtgttcctgttcttcctgtccgtgaccaccggcgtgcactccgaagtgcagctggtggaatctggcggcggactggtgcagcctggcggatctctgagactgtcttgtgccgcctccggcttcaccttctccagctacatgatgagctgggtgcgacaggcccctggcaagggactggaatgggtggccacaatctctggcggaggcgccaacacctactaccccgactctgtgaagggccggttcaccatctctcgggacaacgccaagaactccctgtacctgcagatgaacagcctgcgggccgaggacaccgccgtgtactactgtgcccggcagctgtactacttcgactactggggccagggcaccaccgtgaccgtgtcctctgcttctaccaagggcccctccgtgttccctctggctccttgctccagatccacctccgagtccaccgctgctctgggctgcctcgtgaaggactacttccccgagcctgtgacagtgtcctggaactctggcgccctgacctctggcgtgcacacctttccagcagtgctgcagtcctccggcctgtactccctgtcctccgtcgtgacagtgccctccagctctctgggcaccaagacctacacctgtaacgtggaccacaagccctccaacaccaaggtggacaagagagtggaatctaagtacggccctccctgccccccttgtcctgcccctgaatttctgggcggaccctctgtgtttctgttccccccaaagcccaaggacaccctgatgatctcccggacccccgaagtgacctgcgtggtggtggatgtgtcccaggaagatcccgaggtgcagttcaattggtacgtggacggcgtggaagtgcacaatgccaagaccaagcctagagaggaacagttcaactccacctaccgggtggtgtccgtgctgaccgtgctgcatcaggactggctgaacggcaaagagtacaagtgcaaggtgtccaacaagggcctgcccagctccatcgaaaagaccatctccaaggccaagggccagccccgggaaccccaggtgtacacactgcctccaagccaggaagagatgaccaagaaccaggtgtccctgacctgcctcgtgaaaggcttctacccctccgatatcgccgtggaatgggagtccaacggccagcctgagaacaactacaagaccaccccccctgtgctggactccgacggctccttctttctgtactctcgcctgaccgtggacaagtcccggtggcaggaaggcaacgtgttctcctgcagcgtgatgcacgaggccctgcacaaccactacacccagaagtccctgtccctgtctctgggaaaggccaccaacttctccctgctgaagcaggccggcgacgtggaggagaaccccggccccatgtccgtgcctacccaggtgctgggactgctgctgctgtggctgaccgacgccagatgcgacatccagatgacccagtccccctccagcctgtctgcctctgtgggcgacagagtgaccatcacctgtctggcctcccagaccatcggcacctggctgacctggtatcagcagaagcctggcaaggcccccaagctgctgatctacaccgccaccagtctggccgatggcgtgccctctagattctccggctctggctctggcaccgactttaccctgaccatcagctccctgcagcccgaggacttcgccacctactactgccagcaggtgtactccatcccctggacctttggcggaggcaccaaggtggaaatcaagcggaccgtggccgctccctccgtgttcatcttcccaccttccgacgagcagctgaagtccggaaccgccagtgtcgtgtgcctgctgaacaacttctacccccgcgaggccaaggtgcagtggaaggtggacaacgccctgcagtccggcaactcccaggaatccgtgaccgagcaggactccaaggacagcacctactccctgtcctccaccctgaccctgtccaaggccgactacgagaagcacaaggtgtacgcctgcgaagtgacccaccagggcctgtctagccccgtgaccaagtctttcaaccggggcgagtgctgataagggcccaccggttgataataggctggagcctcggtggccatgcttcttgccccttgggcctccccccagcccctcctccccttcctgcacccgtacccccgtggtctttgaataaagtctgagtgggcggcctcgagccgcggaaaaaaaaaaaaaaaaaaaaaaaaaaaaaagcatatgactaaaaaaaaaaaaaaaaaaaaaaaaaaaaaaaaaaaaaaaaaaaaaaaaaaaaaaaaaaaaaaaaaaaaaattattgtttaaacatttaaattctaga

SEQ ID NO: 124 - DNA, 2602 bp, synthetic construct
  source 1..2602: mol_type = other DNA; note = ACTG1 5'UTR- anti PD-1-CTSB 3'UTR-A30L70 (A1B12- anti PD-1)
ctctcgcactctgttcttccgccgctccgccgtcgcgtttctctgccggtcgcaccaccatggaatggtcctgggtgttcctgttcttcctgtccgtgaccaccggcgtgcactccgaagtgcagctggtggaatctggcggcggactggtgcagcctggcggatctctgagactgtcttgtgccgcctccggcttcaccttctccagctacatgatgagctgggtgcgacaggcccctggcaagggactggaatgggtggccacaatctctggcggaggcgccaacacctactaccccgactctgtgaagggccggttcaccatctctcgggacaacgccaagaactccctgtacctgcagatgaacagcctgcgggccgaggacaccgccgtgtactactgtgcccggcagctgtactacttcgactactggggccagggcaccaccgtgaccgtgtcctctgcttctaccaagggcccctccgtgttccctctggctccttgctccagatccacctccgagtccaccgctgctctgggctgcctcgtgaaggactacttccccgagcctgtgacagtgtcctggaactctggcgccctgacctctggcgtgcacacctttccagcagtgctgcagtcctccggcctgtactccctgtcctccgtcgtgacagtgccctccagctctctgggcaccaagacctacacctgtaacgtggaccacaagccctccaacaccaaggtggacaagagagtggaatctaagtacggccctccctgccccccttgtcctgcccctgaatttctgggcggaccctctgtgtttctgttccccccaaagcccaaggacaccctgatgatctcccggacccccgaagtgacctgcgtggtggtggatgtgtcccaggaagatcccgaggtgcagttcaattggtacgtggacggcgtggaagtgcacaatgccaagaccaagcctagagaggaacagttcaactccacctaccgggtggtgtccgtgctgaccgtgctgcatcaggactggctgaacggcaaagagtacaagtgcaaggtgtccaacaagggcctgcccagctccatcgaaaagaccatctccaaggccaagggccagccccgggaaccccaggtgtacacactgcctccaagccaggaagagatgaccaagaaccaggtgtccctgacctgcctcgtgaaaggcttctacccctccgatatcgccgtggaatgggagtccaacggccagcctgagaacaactacaagaccaccccccctgtgctggactccgacggctccttctttctgtactctcgcctgaccgtggacaagtcccggtggcaggaaggcaacgtgttctcctgcagcgtgatgcacgaggccctgcacaaccactacacccagaagtccctgtccctgtctctgggaaaggccaccaacttctccctgctgaagcaggccggcgacgtggaggagaaccccggccccatgtccgtgcctacccaggtgctgggactgctgctgctgtggctgaccgacgccagatgcgacatccagatgacccagtccccctccagcctgtctgcctctgtgggcgacagagtgaccatcacctgtctggcctcccagaccatcggcacctggctgacctggtatcagcagaagcctggcaaggcccccaagctgctgatctacaccgccaccagtctggccgatggcgtgccctctagattctccggctctggctctggcaccgactttaccctgaccatcagctccctgcagcccgaggacttcgccacctactactgccagcaggtgtactccatcccctggacctttggcggaggcaccaaggtggaaatcaagcggaccgtggccgctccctccgtgttcatcttcccaccttccgacgagcagctgaagtccggaaccgccagtgtcgtgtgcctgctgaacaacttctacccccgcgaggccaaggtgcagtggaaggtggacaacgccctgcagtccggcaactcccaggaatccgtgaccgagcaggactccaaggacagcacctactccctgtcctccaccctgaccctgtccaaggccgactacgagaagcacaaggtgtacgcctgcgaagtgacccaccagggcctgtctagccccgtgaccaagtctttcaaccggggcgagtgctgataagggcccaccggtctgccgtgggcctgtcgtgccagtcctgggggcgagatcgggagaatcacgtcctggaactgcatgttcttgcgactcttgggacttcatcttaacttctcgctgccccagccatgttttcaaccatggcatccctcccccaattagttccctgtcatcctcgtcaaccttctctgtaagtgcctggtaagcttgcccttgcttaagaactcaaaacatagctgtgctctactcgagccgcggaaaaaaaaaaaaaaaaaaaaaaaaaaaaaagcatatgactaaaaaaaaaaaaaaaaaaaaaaaaaaaaaaaaaaaaaaaaaaaaaaaaaaaaaaaaaaaaaaaaaaaaaattattgtttaaacatttaaattctaga

SEQ ID NO: 125 - DNA, 2611 bp, synthetic construct
  source 1..2611: mol_type = other DNA; note = CHCHD10 5'UTR- anti PD-1-CTSB 3'UTR-A30L70 (A15B12- anti PD-1)
ggcatttgtccccgcgacagcaccgctgccgccgtctctaaggtcgcccgggtcccaccgccgccaccatggaatggtcctgggtgttcctgttcttcctgtccgtgaccaccggcgtgcactccgaagtgcagctggtggaatctggcggcggactggtgcagcctggcggatctctgagactgtcttgtgccgcctccggcttcaccttctccagctacatgatgagctgggtgcgacaggcccctggcaagggactggaatgggtggccacaatctctggcggaggcgccaacacctactaccccgactctgtgaagggccggttcaccatctctcgggacaacgccaagaactccctgtacctgcagatgaacagcctgcgggccgaggacaccgccgtgtactactgtgcccggcagctgtactacttcgactactggggccagggcaccaccgtgaccgtgtcctctgcttctaccaagggcccctccgtgttccctctggctccttgctccagatccacctccgagtccaccgctgctctgggctgcctcgtgaaggactacttccccgagcctgtgacagtgtcctggaactctggcgccctgacctctggcgtgcacacctttccagcagtgctgcagtcctccggcctgtactccctgtcctccgtcgtgacagtgccctccagctctctgggcaccaagacctacacctgtaacgtggaccacaagccctccaacaccaaggtggacaagagagtggaatctaagtacggccctccctgccccccttgtcctgcccctgaatttctgggcggaccctctgtgtttctgttccccccaaagcccaaggacaccctgatgatctcccggacccccgaagtgacctgcgtggtggtggatgtgtcccaggaagatcccgaggtgcagttcaattggtacgtggacggcgtggaagtgcacaatgccaagaccaagcctagagaggaacagttcaactccacctaccgggtggtgtccgtgctgaccgtgctgcatcaggactggctgaacggcaaagagtacaagtgcaaggtgtccaacaagggcctgcccagctccatcgaaaagaccatctccaaggccaagggccagccccgggaaccccaggtgtacacactgcctccaagccaggaagagatgaccaagaaccaggtgtccctgacctgcctcgtgaaaggcttctacccctccgatatcgccgtggaatgggagtccaacggccagcctgagaacaactacaagaccaccccccctgtgctggactccgacggctccttctttctgtactctcgcctgaccgtggacaagtcccggtggcaggaaggcaacgtgttctcctgcagcgtgatgcacgaggccctgcacaaccactacacccagaagtccctgtccctgtctctgggaaaggccaccaacttctccctgctgaagcaggccggcgacgtggaggagaaccccggccccatgtccgtgcctacccaggtgctgggactgctgctgctgtggctgaccgacgccagatgcgacatccagatgacccagtccccctccagcctgtctgcctctgtgggcgacagagtgaccatcacctgtctggcctcccagaccatcggcacctggctgacctggtatcagcagaagcctggcaaggcccccaagctgctgatctacaccgccaccagtctggccgatggcgtgccctctagattctccggctctggctctggcaccgactttaccctgaccatcagctccctgcagcccgaggacttcgccacctactactgccagcaggtgtactccatcccctggacctttggcggaggcaccaaggtggaaatcaagcggaccgtggccgctccctccgtgttcatcttcccaccttccgacgagcagctgaagtccggaaccgccagtgtcgtgtgcctgctgaacaacttctacccccgcgaggccaaggtgcagtggaaggtggacaacgccctgcagtccggcaactcccaggaatccgtgaccgagcaggactccaaggacagcacctactccctgtcctccaccctgaccctgtccaaggccgactacgagaagcacaaggtgtacgcctgcgaagtgacccaccagggcctgtctagccccgtgaccaagtctttcaaccggggcgagtgctgataagggcccaccggtctgccgtgggcctgtcgtgccagtcctgggggcgagatcgggagaatcacgtcctggaactgcatgttcttgcgactcttgggacttcatcttaacttctcgctgccccagccatgttttcaaccatggcatccctcccccaattagttccctgtcatcctcgtcaaccttctctgtaagtgcctggtaagcttgcccttgcttaagaactcaaaacatagctgtgctctactcgagccgcggaaaaaaaaaaaaaaaaaaaaaaaaaaaaaagcatatgactaaaaaaaaaaaaaaaaaaaaaaaaaaaaaaaaaaaaaaaaaaaaaaaaaaaaaaaaaaaaaaaaaaaaaattattgtttaaacatttaaattctaga

SEQ ID NO: 126 - DNA, 1653 bp, synthetic construct
  source 1..1653: mol_type = other DNA; note; note (original language) = Nucleotide sequence of firefly luciferase (Fluc)
atggaagacgccaaaaacataaagaaaggcccggcgccattctatccgctggaagatggaaccgctggagagcaactgcataaggctatgaagagatacgccctggttcctggaacaattgcttttacagatgcacatatcgaggtggacatcacttacgctgagtacttcgaaatgtccgttcggttggcagaagctatgaaacgatatgggctgaatacaaatcacagaatcgtcgtatgcagtgaaaactctcttcaattctttatgccggtgttgggcgcgttatttatcggagttgcagttgcgcccgcgaacgacatttataatgaacgtgaattgctcaacagtatgggcatttcgcagcctaccgtggtgttcgtttccaaaaaggggttgcaaaaaattttgaacgtgcaaaaaaagctcccaatcatccaaaaaattattatcatggattctaaaacggattaccagggatttcagtcgatgtacacgttcgtcacatctcatctacctcccggttttaatgaatacgattttgtgccagagtccttcgatagggacaagacaattgcactgatcatgaactcctctggatctactggtctgcctaaaggtgtcgctctgcctcatagaactgcctgcgtgagattctcgcatgccagagatcctatttttggcaatcaaatcattccggatactgcgattttaagtgttgttccattccatcacggttttggaatgtttactacactcggatatttgatatgtggatttcgagtcgtcttaatgtatagatttgaagaagagctgtttctgaggagccttcaggattacaagattcaaagtgcgctgctggtgccaaccctattctccttcttcgccaaaagcactctgattgacaaatacgatttatctaatttacacgaaattgcttctggtggcgctcccctctctaaggaagtcggggaagcggttgccaagaggttccatctgccaggtatcaggcaaggatatgggctcactgagactacatcagctattctgattacacccgagggggatgataaaccgggcgcggtcggtaaagttgttccattttttgaagcgaaggttgtggatctggataccgggaaaacgctgggcgttaatcaaagaggcgaactgtgtgtgagaggtcctatgattatgtccggttatgtaaacaatccggaagcgaccaacgccttgattgacaaggatggatggctacattctggagacatagcttactgggacgaagacgaacacttcttcatcgttgaccgcctgaagtctctgattaagtacaaaggctatcaggtggctcccgctgaattggaatccatcttgctccaacaccccaacatcttcgacgcaggtgtcgcaggtcttcccgacgatgacgccggtgaacttcccgccgccgttgttgttttggagcacggaaagacgatgacggaaaaagagatcgtggattacgtcgccagtcaagtaacaaccgcgaaaaagttgcgcggaggagttgtgtttgtggacgaagtaccgaaaggtcttaccggaaaactcgacgcaagaaaaatcagagagatcctcataaaggccaagaagggcggaaagatcgccgtgtaa

SEQ ID NO: 127 - DNA, 2630 bp, synthetic construct
  source 1..2630: mol_type = other DNA; note; note (original language) = HGF-OS2 expression vector CHCHD10 5'UTR-hHGF-CTSB 3'UTR-A30L70 (A16B12-HGF-OS2)
ccgctgccgccgtctctaaggtcgcccgggtcccaccgccgccaccgctagcgccaccatgtgggtcaccaaactgctgcccgccctgctgctgcagcacgtgctcctgcacctgctgctgctgcctatcgccatcccttacgccgaaggccagagaaagcggagaaataccattcacgaatttaagaagagcgccaagaccacactgatcaagatcgaccctgccctgaaaatcaagaccaagaaagtgaacacagccgaccaatgcgctaatagatgcacaagaaacaaaggcctgcctttcacctgcaaggccttcgtgttcgataaggccagaaagcagtgcctgtggttccccttcaacagcatgagcagcggcgtgaagaaagaattcggtcacgagttcgacctgtacgagaataaggactacattagaaactgcatcatcggcaagggccggagctacaagggcaccgtgagcatcaccaagtctggcatcaagtgccagccatggagttccatgatccctcatgagcacagcttcctgccaagctcttaccggggaaaggatctgcaggagaactattgtagaaatcccagaggcgaggaaggaggaccctggtgttttaccagcaacccagaggtgcggtacgaggtgtgcgacataccccagtgcagcgaggtggaatgcatgacatgcaacggcgagagctaccggggcctgatggaccacacagagagcggcaaaatctgccaaagatgggatcaccagacccctcataggcacaagttcctgcccgagagataccctgacaagggcttcgacgacaattactgccggaaccctgatggacagcctagaccttggtgctacaccctggaccctcacaccagatgggaatactgcgccatcaagacatgtgccgataacaccatgaacgacaccgatgtgccactcgagacaactgagtgtatccagggccagggcgagggctacaggggcaccgtgaacaccatctggaacggcatcccttgtcagcggtgggacagccaatacccccacgaacatgatatgaccccagaaaacttcaagtgcaaagatctgcgggaaaactactgtagaaaccctgacggctccgagagcccttggtgcttcaccaccgaccctaacatcagggtgggctactgtagccagatccccaactgcgacatgagccacggtcaggactgctacagaggaaacggcaagaattacatgggcaacctgagccagaccagaagcggcctgacctgcagcatgtgggacaaaaacatggaagatctgcaccggcacatcttttgggagcctgacgccagcaagctgaatgagaactactgtcggaaccctgacgacgatgctcacggcccttggtgctacacaggcaaccctctgatcccttgggactattgtcctattagcaggtgtgaaggcgacacgacccctacaatcgtgaacctggatcacccagtgatcagctgtgctaaaacaaagcaactgagagtggtgaatggtatcccgacccggaccaacatcggatggatggtcagcctgcggtacagaaacaagcacatctgcggcggtagcctgatcaaggaatcctgggtgttgacagccagacagtgttttcccagcagagatctgaaggactacgaggcctggctgggcatccacgacgtgcacggcagaggcgacgagaagtgcaagcaggttctgaacgtgtcccagctggtgtacggccccgagggctctgatctggttctgatgaagcttgctagacccgctgtgctggatgacttcgtgtccaccatcgacctgccaaattacggatgtacaattcctgaaaagacctcctgttctgtgtacggctggggctacaccggactcatcaactatgacggcctgctgagagtggcccacctgtatatcatgggcaacgagaagtgcagccagcaccatagaggcaaggtgaccctgaacgagtctgaaatctgcgccggagccgagaaaatcggatctggcccctgcgaaggagattacggcggccctctggtctgcgagcagcacaagatgagaatggtgctgggcgtgatcgtgcccggcagaggctgcgccatccctaaccggcctggaatcttcgtgcgcgtggcctattacgccaaatggatccacaaaatcatcctgacatacaaggtcccacagtcttgataagggcccaccggttctgccgtgggcctgtcgtgccagtcctgggggcgagatcgggagaatcacgtcctggaactgcatgttcttgcgactcttgggacttcatcttaacttctcgctgccccagccatgttttcaaccatggcatccctcccccaattagttccctgtcatcctcgtcaaccttctctgtaagtgcctggtaagcttgcccttgcttaagaactcaaaacatagctgtgctctaccgcggaaaaaaaaaaaaaaaaaaaaaaaaaaaaaagcatatgactaaaaaaaaaaaaaaaaaaaaaaaaaaaaaaaaaaaaaaaaaaaaaaaaaaaaaaaaaaaaaaaaaaaaaagtttaaacatttaaattctaga

SEQ ID NO: 128 - RNA, 2187 nt, synthetic construct
  source 1..2187: mol_type = other RNA; note; note (original language) = mRNA sequence of hHGF protein
atgtgggtgaccaaactcctgccagccctgctgctgcagcatgtcctcctgcatctcctcctgctccccatcgccatcccctatgcagagggacaaaggaaaagaagaaatacaattcatgaattcaaaaaatcagcaaagactaccctaatcaaaatagatccagcactgaagataaaaaccaaaaaagtgaatactgcagaccaatgtgctaatagatgtactaggaataaaggacttccattcacttgcaaggcttttgtttttgataaagcaagaaaacaatgcctctggttccccttcaatagcatgtcaagtggagtgaaaaaagaatttggccatgaatttgacctctatgaaaacaaagactacattagaaactgcatcattggtaaaggacgcagctacaagggaacagtatctatcactaagagtggcatcaaatgtcagccctggagttccatgataccacacgaacacagctttttgccttcgagctatcggggtaaagacctacaggaaaactactgtcgaaatcctcgaggggaagaagggggaccctggtgtttcacaagcaatccagaggtacgctacgaagtctgtgacattcctcagtgttcagaagttgaatgcatgacctgcaatggggagagttatcgaggtctcatggatcatacagaatcaggcaagatttgtcagcgctgggatcatcagacaccacaccggcacaaattcttgcctgaaagatatcccgacaagggctttgatgataattattgccgcaatcccgatggccagccgaggccatggtgctatactcttgaccctcacacccgctgggagtactgtgcaattaaaacatgcgctgacaatactatgaatgacactgatgttcctttggaaacaactgaatgcatccaaggtcaaggagaaggctacaggggcactgtcaataccatttggaatggaattccatgtcagcgttgggattctcagtatcctcacgagcatgacatgactcctgaaaatttcaagtgcaaggacctacgagaaaattactgccgaaatccagatgggtctgaatcaccctggtgttttaccactgatccaaacatccgagttggctactgctcccaaattccaaactgtgatatgtcacatggacaagattgttatcgtgggaatggcaaaaattatatgggcaacttatcccaaacaagatctggactaacatgttcaatgtgggacaagaacatggaagacttacatcgtcatatcttctgggaaccagatgcaagtaagctgaatgagaattactgccgaaatccagatgatgatgctcatggaccctggtgctacacgggaaatccactcattccttgggattattgccctatttctcgttgtgaaggtgataccacacctacaatagtcaatttagaccatcccgtaatatcttgtgccaaaacgaaacaattgcgagttgtaaatgggattccaacacgaacaaacataggatggatggttagtttgagatacagaaataaacatatctgcggaggatcattgataaaggagagttgggttcttactgcacgacagtgtttcccttctcgagacttgaaagattatgaagcttggcttggaattcatgatgtccacggaagaggagatgagaaatgcaaacaggttctcaatgtttcccagctggtatatggccctgaaggatcagatctggttttaatgaagcttgccaggcctgctgtcctggatgattttgttagtacgattgatttacctaattatggatgcacaattcctgaaaagaccagttgcagtgtttatggctggggctacactggattgatcaactatgatggcctattacgagtggcacatctctatataatgggaaatgagaaatgcagccagcatcatcgagggaaggtgactctgaatgagtctgaaatatgtgctggggctgaaaagattggatcaggaccatgtgagggggattatggtggcccacttgtttgtgagcaacataaaatgagaatggttcttggtgtcattgttcctggtcgtggatgtgccattccaaatcgtcctggtatttttgtccgagtagcatattatgcaaaatggatacacaaaattattttaacatataaggtaccacagtcatag

SEQ ID NO: 129 - RNA, 2187 nt, synthetic construct
  source 1..2187: mol_type = other RNA; note; note (original language) = hHGF codon-optimized mRNA sequence 1 (hHGF-OS1)
atgtgggtgaccaaactgctccccgctctgctgctgcagcatgtgctgctccacctgctgctgctgccaatcgccatcccctacgctgaaggacagcggaagcgcagaaacacaattcacgaattcaagaagtccgccaaaacaacactgatcaagatcgaccctgccctgaaaatcaaaaccaagaaggtgaacactgccgatcagtgcgccaacagatgcacaagaaacaaaggcctgcccttcacatgcaaggcctttgtgttcgacaaggccagaaagcagtgcctgtggttccctttcaacagcatgagctctggcgtgaagaaagagttcggccacgaattcgacctgtacgagaacaaggattacatcagaaattgtatcatcggcaagggcagaagctacaaaggcacagtgtccatcaccaaaagcggcattaagtgtcagccttggagcagcatgatccctcacgagcacagcttcctgcctagctcttacagaggcaaggacctgcaggagaattactgccggaaccctagaggcgaggaaggcggcccttggtgctttaccagcaaccctgaggtgcggtacgaggtgtgtgacatcccccagtgcagcgaagtggaatgcatgacctgtaatggcgagagctacagaggcctcatggaccatacagagagcggaaagatttgtcaaagatgggatcaccagacacctcacagacacaaattcctgcccgaaagatatcctgacaagggcttcgacgacaactactgcagaaatcctgatggccaacccagaccttggtgctacaccctggatcctcataccagatgggagtactgtgccatcaagacctgcgctgataataccatgaacgacaccgatgtgcctctggaaacaaccgagtgcatccagggacagggcgaaggctaccggggcaccgtgaacaccatctggaacggcatcccctgccagagatgggacagccagtacccccacgaacacgatatgacccctgagaacttcaagtgcaaggacctgagagaaaattactgcagaaacccagacggaagcgagtctccttggtgttttaccaccgaccccaacatccgggtgggttactgcagccaaatccccaattgcgacatgagccacggccaggactgctaccggggaaacggcaaaaactacatgggcaatctgagccagacccggagcggtctgacctgctccatgtgggataagaacatggaagatctgcaccggcacatcttctgggagcctgacgcttctaagctgaacgagaactactgtaggaacccagacgacgatgcccacggtccctggtgctacaccggcaacccgctgatcccttgggactattgtcctatcagccgctgcgagggcgatacaacacctaccatcgtgaacctggaccaccctgtgatctcttgcgccaagaccaagcagctgagagtggtgaacggcatcccaacacggaccaacatcggatggatggtctccctgagataccggaacaagcacatctgcggcggctctctgatcaaggaatcttgggtcctgaccgccagacagtgcttccccagccgggacctgaaggactatgaggcctggctgggaatccacgacgtgcacggcagaggcgacgagaagtgcaagcaagtgctgaacgtgtcccagctggtgtacggccctgagggatctgatctggtcctgatgaaactggccagacccgccgtgctggacgactttgtgtccaccatcgacctgcctaactacggctgcaccatccctgaaaagaccagctgcagcgtgtacggctggggctatacaggcctgatcaactacgacggtctgctgcgggttgctcacctgtacatcatgggcaacgagaagtgcagccagcaccacagaggaaaggttacacttaacgagagcgagatctgcgccggcgccgagaaaatcggctccggcccttgtgaaggcgactacggaggccctctggtgtgcgaacagcacaagatgagaatggtgctgggcgtgatcgtgcccggaagaggctgtgcaatccctaataggcccggcattttcgtgcgggtggcctactacgccaagtggatccacaagatcatcctgacgtacaaggtgcctcagagctga

SEQ ID NO: 130 - RNA, 2187 nt, synthetic construct
  source 1..2187: mol_type = other RNA; note; note (original language) = hHGF codon-optimized mRNA sequence 2 (hHGF-OS2)
atgtgggtcaccaaactgctgcccgccctgctgctgcagcacgtgctcctgcacctgctgctgctgcctatcgccatcccttacgccgaaggccagagaaagcggagaaataccattcacgaatttaagaagagcgccaagaccacactgatcaagatcgaccctgccctgaaaatcaagaccaagaaagtgaacacagccgaccaatgcgctaatagatgcacaagaaacaaaggcctgcctttcacctgcaaggccttcgtgttcgataaggccagaaagcagtgcctgtggttccccttcaacagcatgagcagcggcgtgaagaaagaattcggtcacgagttcgacctgtacgagaataaggactacattagaaactgcatcatcggcaagggccggagctacaagggcaccgtgagcatcaccaagtctggcatcaagtgccagccatggagttccatgatccctcatgagcacagcttcctgccaagctcttaccggggaaaggatctgcaggagaactattgtagaaatcccagaggcgaggaaggaggaccctggtgttttaccagcaacccagaggtgcggtacgaggtgtgcgacataccccagtgcagcgaggtggaatgcatgacatgcaacggcgagagctaccggggcctgatggaccacacagagagcggcaaaatctgccaaagatgggatcaccagacccctcataggcacaagttcctgcccgagagataccctgacaagggcttcgacgacaattactgccggaaccctgatggacagcctagaccttggtgctacaccctggaccctcacaccagatgggaatactgcgccatcaagacatgtgccgataacaccatgaacgacaccgatgtgccactcgagacaactgagtgtatccagggccagggcgagggctacaggggcaccgtgaacaccatctggaacggcatcccttgtcagcggtgggacagccaatacccccacgaacatgatatgaccccagaaaacttcaagtgcaaagatctgcgggaaaactactgtagaaaccctgacggctccgagagcccttggtgcttcaccaccgaccctaacatcagggtgggctactgtagccagatccccaactgcgacatgagccacggtcaggactgctacagaggaaacggcaagaattacatgggcaacctgagccagaccagaagcggcctgacctgcagcatgtgggacaaaaacatggaagatctgcaccggcacatcttttgggagcctgacgccagcaagctgaatgagaactactgtcggaaccctgacgacgatgctcacggcccttggtgctacacaggcaaccctctgatcccttgggactattgtcctattagcaggtgtgaaggcgacacgacccctacaatcgtgaacctggatcacccagtgatcagctgtgctaaaacaaagcaactgagagtggtgaatggtatcccgacccggaccaacatcggatggatggtcagcctgcggtacagaaacaagcacatctgcggcggtagcctgatcaaggaatcctgggtgttgacagccagacagtgttttcccagcagagatctgaaggactacgaggcctggctgggcatccacgacgtgcacggcagaggcgacgagaagtgcaagcaggttctgaacgtgtcccagctggtgtacggccccgagggctctgatctggttctgatgaagcttgctagacccgctgtgctggatgacttcgtgtccaccatcgacctgccaaattacggatgtacaattcctgaaaagacctcctgttctgtgtacggctggggctacaccggactcatcaactatgacggcctgctgagagtggcccacctgtatatcatgggcaacgagaagtgcagccagcaccatagaggcaaggtgaccctgaacgagtctgaaatctgcgccggagccgagaaaatcggatctggcccctgcgaaggagattacggcggccctctggtctgcgagcagcacaagatgagaatggtgctgggcgtgatcgtgcccggcagaggctgcgccatccctaaccggcctggaatcttcgtgcgcgtggcctattacgccaaatggatccacaaaatcatcctgacatacaaggtcccacagtcttga

SEQ ID NO: 131 - RNA, 2187 nt, synthetic construct
  source 1..2187: mol_type = other RNA; note; note (original language) = hHGF codon-optimized mRNA sequence 3 (hHGF-OS3)
atgtgggtgaccaagctgctgcccgccctgctcctgcagcacgtgctgctgcacctgctcctgctgcccatcgccatcccctacgccgaggggcagagaaagagaagaaacaccatccacgagttcaagaagagcgccaagaccaccctgatcaagatcgaccccgccctgaagatcaagaccaagaaggtgaacaccgccgatcagtgcgccaacagatgcacaagaaacaagggcctgcccttcacctgcaaggccttcgtgttcgacaaggctagaaagcagtgcctgtggttccccttcaacagcatgagcagcggcgtgaagaaggagttcggccacgagttcgacctgtacgagaacaaggactacatcagaaactgcatcatcggcaagggcagaagctacaagggcaccgtgagcatcaccaagagcggcatcaagtgtcagccctggagcagcatgatcccccatgagcacagcttcctgcctagcagctacagagggaaggacctgcaagagaactactgcagaaaccctagaggcgaggagggcggcccttggtgtttcacaagcaatcccgaggtgagatacgaggtgtgcgacatccctcagtgcagcgaggtggagtgcatgacctgcaacggcgaaagctatagaggcctgatggaccacaccgagagcggcaagatttgtcagcggtgggatcaccaaaccccccacagacacaagttcctgcccgagagataccccgacaagggcttcgacgacaattactgtagaaaccccgacgggcagcctagaccctggtgttacaccctggacccccacacaagatgggagtactgcgccatcaagacctgcgccgacaacaccatgaacgacaccgacgtgcccctggagaccaccgagtgcatccaaggccaaggcgagggctacagaggcaccgtgaacaccatctggaacggcattccctgtcagagatgggacagccaatacccccatgaacacgatatgacccccgagaacttcaagtgcaaggacctgagagagaactactgccggaaccccgatggcagcgaatccccttggtgcttcaccaccgaccccaacatcagagtgggctactgcagccaaatccccaactgcgacatgagccacggccaagactgttacagagggaacggcaagaactacatgggcaacctgagccaaacaagaagcggcctgacctgcagcatgtgggacaagaacatggaggacctgcacagacacatcttctgggagcccgacgctagcaagctgaacgagaactactgtcggaaccccgacgacgatgcccacggcccctggtgctacaccggcaaccccctgatcccctgggactactgccccatcagcagatgcgagggcgacaccacccccaccatcgtgaacctggaccaccccgtgatcagctgtgccaagaccaagcaactgagagtggtgaacggcatccccacaagaaccaacattggctggatggtgagcctgagatacagaaacaagcacatctgcggcggcagcctgatcaaggagagctgggtgctgaccgctagacagtgcttccctagcagagacctgaaggactacgaggcctggctgggcatccacgacgtgcacggcagaggcgacgagaagtgtaaacaagtgctgaacgtgagccaactggtgtacggccccgagggcagcgacctggtgctgatgaagctggctagacccgccgtgctggacgacttcgtgagcaccatcgacctgcccaactacggctgcaccatccccgagaagacaagctgcagcgtgtacggctggggctacaccggcctgatcaactacgacggcctgctgagagtggcccacctgtacatcatgggcaacgagaagtgcagccaacaccaccggggcaaagtgaccctgaacgagagcgagatctgcgccggggctgagaaaatcggcagcggcccctgcgagggggactacgggggccccctggtgtgcgagcagcacaagatgagaatggtgctgggcgtgatcgtgcccggcagaggctgcgccatccccaacagacccggcatcttcgtgagagtggcctactacgccaagtggatccacaagatcatcctgacctacaaggtgcctcagagctga

SEQ ID NO: 132 - RNA, 2626 nt, synthetic construct
  source 1..2626: mol_type = other RNA; note; note (original language) = CHCHD10 5'UTR- hHGF-CTSB 3'UTR-A120
agggaagcttccgctgccgccgtctctaaggtcgcccgggtcccaccgccgccaccgccgccaccatgtgggtcaccaaactgctgcccgccctgctgctgcagcacgtgctcctgcacctgctgctgctgcctatcgccatcccttacgccgaaggccagagaaagcggagaaataccattcacgaatttaagaagagcgccaagaccacactgatcaagatcgaccctgccctgaaaatcaagaccaagaaagtgaacacagccgaccaatgcgctaatagatgcacaagaaacaaaggcctgcctttcacctgcaaggccttcgtgttcgataaggccagaaagcagtgcctgtggttccccttcaacagcatgagcagcggcgtgaagaaagaattcggtcacgagttcgacctgtacgagaataaggactacattagaaactgcatcatcggcaagggccggagctacaagggcaccgtgagcatcaccaagtctggcatcaagtgccagccatggagttccatgatccctcatgagcacagcttcctgccaagctcttaccggggaaaggatctgcaggagaactattgtagaaatcccagaggcgaggaaggaggaccctggtgttttaccagcaacccagaggtgcggtacgaggtgtgcgacataccccagtgcagcgaggtggaatgcatgacatgcaacggcgagagctaccggggcctgatggaccacacagagagcggcaaaatctgccaaagatgggatcaccagacccctcataggcacaagttcctgcccgagagataccctgacaagggcttcgacgacaattactgccggaaccctgatggacagcctagaccttggtgctacaccctggaccctcacaccagatgggaatactgcgccatcaagacatgtgccgataacaccatgaacgacaccgatgtgccactcgagacaactgagtgtatccagggccagggcgagggctacaggggcaccgtgaacaccatctggaacggcatcccttgtcagcggtgggacagccaatacccccacgaacatgatatgaccccagaaaacttcaagtgcaaagatctgcgggaaaactactgtagaaaccctgacggctccgagagcccttggtgcttcaccaccgaccctaacatcagggtgggctactgtagccagatccccaactgcgacatgagccacggtcaggactgctacagaggaaacggcaagaattacatgggcaacctgagccagaccagaagcggcctgacctgcagcatgtgggacaaaaacatggaagatctgcaccggcacatcttttgggagcctgacgccagcaagctgaatgagaactactgtcggaaccctgacgacgatgctcacggcccttggtgctacacaggcaaccctctgatcccttgggactattgtcctattagcaggtgtgaaggcgacacgacccctacaatcgtgaacctggatcacccagtgatcagctgtgctaaaacaaagcaactgagagtggtgaatggtatcccgacccggaccaacatcggatggatggtcagcctgcggtacagaaacaagcacatctgcggcggtagcctgatcaaggaatcctgggtgttgacagccagacagtgttttcccagcagagatctgaaggactacgaggcctggctgggcatccacgacgtgcacggcagaggcgacgagaagtgcaagcaggttctgaacgtgtcccagctggtgtacggccccgagggctctgatctggttctgatgaagcttgctagacccgctgtgctggatgacttcgtgtccaccatcgacctgccaaattacggatgtacaattcctgaaaagacctcctgttctgtgtacggctggggctacaccggactcatcaactatgacggcctgctgagagtggcccacctgtatatcatgggcaacgagaagtgcagccagcaccatagaggcaaggtgaccctgaacgagtctgaaatctgcgccggagccgagaaaatcggatctggcccctgcgaaggagattacggcggccctctggtctgcgagcagcacaagatgagaatggtgctgggcgtgatcgtgcccggcagaggctgcgccatccctaaccggcctggaatcttcgtgcgcgtggcctattacgccaaatggatccacaaaatcatcctgacatacaaggtcccacagtcttgaaccggttctgccgtgggcctgtcgtgccagtcctgggggcgagatcgggagaatcacgtcctggaactgcatgttcttgcgactcttgggacttcatcttaacttctcgctgccccagccatgttttcaaccatggcatccctcccccaattagttccctgtcatcctcgtcaaccttctctgtaagtgcctggtaagcttgcccttgcttaagaactcaaaacatagctgtgctctaccgcggaaaaaaaaaaaaaaaaaaaaaaaaaaaaaaaaaaaaaaaaaaaaaaaaaaaaaaaaaaaaaaaaaaaaaaaaaaaaaaaaaaaaaaaaaaaaaaaaaaaaaaaaaaaaaaaaaaaaaaaattatttctag